European Patent Specification EP 3 601 330 B1, published November 13, 2024. Title: CHIMERIC POLYPEPTIDES AND METHODS OF ALTERING THE MEMBRANE LOCALIZATION OF THE SAME. Applicant: Cell Design Labs, Inc. The sequence listing filed with the application follows.

SEQUENCE LISTING (119 sequences)

SEQ ID NO: 1 - protein, 220 aa, Homo sapiens
MLRLLLALNLFPSIQVTGNKILVKQSPMLVAYDNAVNLSCKYSYNLFSREFRASLHKGLDSAVEVCVVYGNYSQQLQVYSKTGFNCDGKLGNESVTFYLQNLYVNQTDIYFCKIEVMYPPPYLDNEKSNGTIIHVKGKHLCPSPLFPGPSKPFWVLVVVGGVLACYSLLVTVAFIIFWVRSKRSRLLHSDYMNMTPRRPGPTRKHYQPYAPPRDFAAYRS

SEQ ID NO: 2 - protein, 164 aa, Homo sapiens
MKWKALFTAAILQAQLPITEAQSFGLLDPKLCYLLDGILFIYGVILTALFLRVKFSRSADAPAYQQGQNQLYNELNLGRREEYDVLDKRRGRDPEMGGKPQRRKNPQEGLYNELQKDKMAEAYSEIGMKGERRRGKGHDGLYQGLSTATKDTYDALHMQALPPR

SEQ ID NO: 3 - protein, 23 aa, Homo sapiens
LGLLVAGVLVLLVSLGVAIHLCC

SEQ ID NO: 4 - protein, 26 aa, Homo sapiens
VAAILGLGLVLGLLGPLAILLALYLL

SEQ ID NO: 5 - protein, 25 aa, Homo sapiens
ALIVLGGVAGLLLFIGLGIFFCVRC

SEQ ID NO: 6 - protein, 23 aa, Homo sapiens
LCYLLDGILFIYGVILTALFLRV

SEQ ID NO: 7 - protein, 26 aa, Homo sapiens
WVLVVVGGVLACYSLLVTVAFIIFWV

SEQ ID NO: 8 - protein, 24 aa, Homo sapiens
IYIWAPLAGTCGVLLLSLVITLYC

SEQ ID NO: 9 - protein, 24 aa, Homo sapiens
ALPAALAVISFLLGLGLGVACVLA

SEQ ID NO: 10 - protein, 250 aa, Homo sapiens
SKKNSLALSLTADQMVSALLDAEPPILYSEYDPTRPFSEASMMGLLTNLADRELVHMINWAKRVPGFVDLTLHDQVHLLECAWLEILMIGLVWRSMEHPGKLLFAPNLLLDRNQGKCVEGMVEIFDMLLATSSRFRMMNLQGEEFVCLKSIILLNSGVYTFLSSTLKSLEEKDHIHRVLDKITDTLIHLMAKAGLTLQQQHQRLAQLLLILSHIRHMSNKGMEHLYSMKCKNVVPLYDLLLEMLDAHRLH

SEQ ID NO: 11 - protein, 248 aa, Homo sapiens
ALSLTADQMVSALLDAEPPILYSEYDPTRPFSEASMMGLLTNLADRELVHMINWAKRVPGFVDLTLHDQVHLLECAWLEILMIGLVWRSMEHPGKLLFAPNLLLDRNQGKCVEGMVEIFDMLLATSSRFRMMNLQGEEFVCLKSIILLNSGVYTFLSSTLKSLEEKDHIHRVLDKITDTLIHLMAKAGLTLQQQHQRLAQLLLILSHIRHMSNKGMEHLYSMKCKNVVPLYDLLLEMLDAHRLHAPTS

SEQ ID NO: 12 - protein, 200 aa, Homo sapiens
SPGQDIQLIPPLINLLMSIEPDVIYAGHDNTKPDTSSSLLTSLNQLGERQLLSVVKWSKSLPGFRNLHIDDQITLIQYSWMSLMVFGLGWRSYKHVSGQMLYFAPDLILNEQRMKESSFYSLCLTMWQIPQEFVKLQVSQEEFLCMKVLLLLNTIPLEGLRSQTQFEEMRSSYIRELIKAIGLRQKGVVSSSQRFYQLTK

SEQ ID NO: 13 - protein, 261 aa, Homo sapiens
FTFSPGQDIQLIPPLINLLMSIEPDVIYAGHDNTKPDTSSSLLTSLNQLGERQLLSVVKWSKSLPGFRNLHIDDQITLIQYSWMSLMVFGLGWRSYKHVSGQMLYFAPDLILNEQRMKESSFYSLCLTMWQIPQEFVKLQVSQEEFLCMKVLLLLNTIPLEGLRSQTQFEEMRSSYIRELIKAIGLRQKGVVSSSQRFYQLTKLLDNLHDLVKQLHLYCLNTFIQSRALSVEFPEMMSEVIAAQLPKILAGMVKPLLFHKK

SEQ ID NO: 14 - protein, 249 aa, Homo sapiens
PIFLNVLEAIEPGVVCAGHDNNQPDSFAALLSSLNELGERQLVHVVKWAKALPGFRNLHVDDQMAVIQYSWMGLMVFAMGWRSFTNVNSRMLYFAPDLVFNEYRMHKSRMYSQCVRMRHLSQEFGWLQITPQEFLCMKALLLFSIIPVDGLKNQKFFDELRMNYIKELDRIIACKRKNPTSCSRRFYQLTKLLDSVQPIARELHQFTFDLLIKSHMVSVDFPEMMAEIISVQVPKILSGKVKPIYFHTQ

SEQ ID NO: 15 - protein, 283 aa, Homo sapiens
SLEEGEASSTTSPTEETTQKLTVSHIEGYECQPIFLNVLEAIEPGVVCAGHDNNQPDSFAALLSSLNELGERQLVHVVKWAKALPGFRNLHVDDQMAVIQYSWMGLMVFAMGWRSFTNVNSRMLYFAPDLVFNEYRMHKSRMYSQCVRMRHLSQEFGWLQITPQEFLCMKALLLFSIIPVDGLKNQKFFDELRMNYIKELDRIIACKRKNPTSCSRRFYQLTKLLDSVQPIARELHQFTFDLLIKSHMVSVDFPEMMAEIISVQVPKILSGKVKPIYFHTQEG

SEQ ID NO: 16 - protein, 266 aa, Homo sapiens
ETTQKLTVSHIEGYECQPIFLNVLEAIEPGVVCAGHDNNQPDSFAALLSSLNELGERQLVHVVKWAKALPGFRNLHVDDQMAVIQYSWMGLMVFAMGWRSFTNVNSRMLYFAPDLVFNEYRMHKSRMYSQCVRMRHLSQEFGWLQITPQEFLCMKALLLFSIIPVDGLKNQKFFDELRMNYIKELDRIIACKRKNPTSCSRRFYQLTKLLDSVQPIARELHQFTFDLLIKSHMVSVDFPEMMAEIISVQVPKILSGKVKPIYFHTQ

SEQ ID NO: 17 - protein, 164 aa, Homo sapiens; identical to SEQ ID NO: 2

SEQ ID NO: 18 - protein, 220 aa, Homo sapiens; identical to SEQ ID NO: 1

SEQ ID NO: 19 - protein, 255 aa, Homo sapiens
MGNSCYNIVATLLLVLNFERTRSLQDPCSNCPAGTFCDNNRNQICSPCPPNSFSSAGGQRTCDICRQCKGVFRTRKECSSTSNAECDCTPGFHCLGAGCSMCEQDCKQGQELTKKGCKDCCFGTFNDQKRGICRPWTNCSLDGKSVLVNGTKERDVVCGPSPADLSPGASSVTPPAPAREPGHSPQIISFFLALTSTALLFLLFFLTLRFSVVKRGRKKLLYIFKQPFMRPVQTTQEEDGCSCRFPEEEEGGCEL

SEQ ID NO: 20 - protein, 10 aa, Artificial Sequence
  Linker sequence
GSGSGSGSGS

SEQ ID NO: 21 - protein, 8 aa, Artificial Sequence
  Linker sequence
GSGSGSGS

SEQ ID NO: 22 - protein, 8 aa, Artificial Sequence
  Linker sequence
RSGSGSGS

SEQ ID NO: 23 - protein, 8 aa, Artificial Sequence
  Linker sequence
GSGSGSGS

SEQ ID NO: 24 - DNA, 30 bp, Artificial Sequence
  Linker sequence
ggatccggcagcggatctggcagtggaagc

SEQ ID NO: 25 - DNA, 24 bp, Artificial Sequence
  Linker sequence
ggatctggctctggaagcggcagc

SEQ ID NO: 26 - DNA, 24 bp, Artificial Sequence
  Linker sequence
agatccggatctggaagtggctcc

SEQ ID NO: 27 - DNA, 24 bp, Artificial Sequence
  Linker sequence
ggaagtggatctgggagcggctct

SEQ ID NO: 28 - protein, 297 aa, Homo sapiens
DRRGGRMLKHKRQRDDGEGRGEVGSAGDMRAANLWPSPLMIKRSKKNSLALSLTADQMVSALLDAEPPILYSEYDPTRPFSEASMMGLLTNLADRELVHMINWAKRVPGFVDLTLHDQVHLLECAWLEILMIGLVWRSMEHPGKLLFAPNLLLDRNQGKCVEGMVEIFDMLLATSSRFRMMNLQGEEFVCLKSIILLNSGVYTFLSSTLKSLEEKDHIHRVLDKITDTLIHLMAKAGLTLQQQHQRLAQLLLILSHIRHMSNKRMEHLYSMKCKNVVPLFDLLLEMLDAHRLHAPTS

SEQ ID NO: 29 - protein, 256 aa, Homo sapiens
GQDIQLIPPLINLLMSIEPDVIYAGHDNTKPDTSSSLLTSLNQLGERQLLSVVKWSKSLPGFRNLHIDDQITLIQYSWMSLMVFGLGWRSYKHVSGQMLYFAPDLILNEQRMKESSFYSLCLTMWQIPQEFVKLQVSQEEFLCMKVLLLLNTIPLEGLRSQTQFEEMRSSYIRELIKAIGLRQKGVVSSSQRFYQLTKLLDNLHDLVKQLHLYCLNTFIQSRALSVEFPEMMSEVIAAQLPKILAGMVKPLLFHKK

SEQ ID NO: 30 - DNA, 3183 bp, Artificial Sequence
  v.2 construct
atggctctgcctgtgacagctctgctgctgcctctggccctgctgctgcatgccgctagacctgagcagaagctgatctccgaagaggacctggacatccagatgacccagaccaccagcagcctgagcgccagcctgggcgatagagtgaccatcagctgcagagccagccaggacatcagcaagtacctgaactggtatcagcagaaacccgacggcaccgtgaagctgctgatctaccacaccagcagactgcacagcggcgtgcccagcagattttctggcagcggctccggcaccgactacagcctgaccatctccaacctggaacaggaagatatcgctacctacttctgtcagcaaggcaacaccctgccctacaccttcggcggaggcaccaagctggaaatcacaggcggcggaggatctggcggaggcggaagtggcggagggggatctgaagtgaaactgcaggaaagcggccctggcctggtggccccatctcagtctctgagcgtgacctgtaccgtgtccggcgtgtccctgcctgactatggcgtgtcctggatcagacagccccccagaaagggcctggaatggctgggagtgatctggggcagcgagacaacctactacaacagcgccctgaagtcccggctgaccatcatcaaggacaactccaagagccaggtgttcctgaagatgaacagcctgcagaccgacgacaccgccatctactactgcgccaagcactactactacggcggcagctacgccatggactactggggccagggcacaagcgtgaccgtgtctagcacaaccacccctgcccctagacctccaaccccagcccctacaatcgccagccagcctctgtctctgaggcccgaggcttgtagaccagctgctggcggagccgtgcacaccagaggactggatttcgcctgcgacatctacatctgggcccctctggccggcacatgtggcgtgctgctgctgagcctcgtgatcaccctgtactgcggatccaagcggggcagaaagaaactgctgtacatctttaagcagcccttcatgcggcccgtgcagaccacccaggaagaggacggctgctcctgcagattccccgaggaagaagaaggcggctgcgagctgggcagcggatctggcagtggaagcgatagaagaggcggcagaatgctgaaacacaagcggcagagggacgacggggaaggcagaggcgaagtgggatctgccggcgatatgagagccgccaacctgtggcctagccccctgatgatcaagcggagcaagaagaactccctggccctgagcctgaccgccgaccagatggtgtctgccctgctggatgccgagccccccatcctgtacagcgagtacgaccccaccagacccttcagcgaggccagcatgatgggcctgctgaccaacctggccgaccgggaactggtgcacatgatcaactgggccaagcgggtgcccggcttcgtggatctgacactgcacgaccaggtgcacctgctggaatgcgcttggctggaaatcctgatgatcggcctcgtgtggcggagcatggaacaccctggcaagctgctgttcgcccccaacctgctgctggaccggaaccagggcaaatgcgtggaaggcatggtggaaatcttcgacatgctgctggccacctccagccggttccggatgatgaacctgcagggcgaagagttcgtgtgtctgaagtccatcatcctgctgaatagcggcgtgtacaccttcctgagcagcaccctgaaaagcctggaagaaaaggaccacatccaccgggtgctggacaagatcaccgacaccctgattcacctgatggccaaggccggactgaccctgcagcagcagcatcagagactggctcagctgctgctgatcctgtcccacatccggcacatgagcaacaagcggatggaacatctgtacagcatgaagtgcaagaacgtggtgcctctgttcgatctgctgctggaaatgctggacgcccacaggctgcacgccccaacatccagatccggatctggaagtggctccctgagagtgaagtttagcagaagcgccgacgcccctgcctatcagcagggacagaaccagctgtataacgagctgaacctgggcaggcgggaagagtacgacgtgctggataagaggcggggcagggaccctgaaatgggcggcaaacccagacggaagaacccccaggaaggcctgtacaacgaactgcagaaagacaagatggccgaggcctacagcgagatcggaatgaagggcgagcggcggagaggcaagggacatgatggcctgtaccagggcctgtccaccgccaccaaggacacctatgacgccctgcacatgcaggccctgcctccaagaggaagtggatctgggagcggctctatggtgtctaagggggaagaggacaacatggccatcatcaaagaattcatgcggttcaaggtgcacatggaaggctccgtgaatggccacgaattcgagatcgagggggagggcgagggcagaccttatgagggaacccagaccgccaagctgaaagtgaccaagggcggacccctgcctttcgcctgggatatcctgtctccccagtttatgtacggcagcaaggcctacgtgaagcaccccgccgacatccccgactacctgaagctgagcttccctgagggcttcaagtgggagagagtgatgaatttcgaggacggcggagtcgtgacagtgacccaggatagctctctgcaggacggcgagttcatctacaaagtgaagctgcggggcaccaacttccccagcgacggacccgtgatgcagaaaaagaccatgggctgggaggccagctccgagagaatgtacccagaggacggggccctgaagggggagatcaagcagcggctgaaactgaaggatggcggccactacgacgcagaagtgaaaaccacctacaaggccaagaaacctgtgcagctgcctggcgcctacaatgtgaacatcaagctggacattaccagccacaacgaggactacaccatcgtggaacagtacgagcgggccgagggcaggcattctacaggcggaatggatgaactgtataagtgcgtgaccgactag

SEQ ID NO: 31 - protein, 1060 aa, Artificial Sequence
  v.2 construct
MALPVTALLLPLALLLHAARPEQKLISEEDLDIQMTQTTSSLSASLGDRVTISCRASQDISKYLNWYQQKPDGTVKLLIYHTSRLHSGVPSRFSGSGSGTDYSLTISNLEQEDIATYFCQQGNTLPYTFGGGTKLEITGGGGSGGGGSGGGGSEVKLQESGPGLVAPSQSLSVTCTVSGVSLPDYGVSWIRQPPRKGLEWLGVIWGSETTYYNSALKSRLTIIKDNSKSQVFLKMNSLQTDDTAIYYCAKHYYYGGSYAMDYWGQGTSVTVSSTTTPAPRPPTPAPTIASQPLSLRPEACRPAAGGAVHTRGLDFACDIYIWAPLAGTCGVLLLSLVITLYCGSKRGRKKLLYIFKQPFMRPVQTTQEEDGCSCRFPEEEEGGCELGSGSGSGSDRRGGRMLKHKRQRDDGEGRGEVGSAGDMRAANLWPSPLMIKRSKKNSLALSLTADQMVSALLDAEPPILYSEYDPTRPFSEASMMGLLTNLADRELVHMINWAKRVPGFVDLTLHDQVHLLECAWLEILMIGLVWRSMEHPGKLLFAPNLLLDRNQGKCVEGMVEIFDMLLATSSRFRMMNLQGEEFVCLKSIILLNSGVYTFLSSTLKSLEEKDHIHRVLDKITDTLIHLMAKAGLTLQQQHQRLAQLLLILSHIRHMSNKRMEHLYSMKCKNVVPLFDLLLEMLDAHRLHAPTSRSGSGSGSLRVKFSRSADAPAYQQGQNQLYNELNLGRREEYDVLDKRRGRDPEMGGKPRRKNPQEGLYNELQKDKMAEAYSEIGMKGERRRGKGHDGLYQGLSTATKDTYDALHMQALPPRGSGSGSGSMVSKGEEDNMAIIKEFMRFKVHMEGSVNGHEFEIEGEGEGRPYEGTQTAKLKVTKGGPLPFAWDILSPQFMYGSKAYVKHPADIPDYLKLSFPEGFKWERVMNFEDGGVVTVTQDSSLQDGEFIYKVKLRGTNFPSDGPVMQKKTMGWEASSERMYPEDGALKGEIKQRLKLKDGGHYDAEVKTTYKAKKPVQLPGAYNVNIKLDITSHNEDYTIVEQYERAEGRHSTGGMDELYKCVTD

SEQ ID NO: 32 - DNA, 3183 bp, Artificial Sequence
  v.3 construct
atggctctgcctgtgacagctctgctgctgcctctggccctgctgctgcatgccgctagacctgagcagaagctgatctccgaagaggacctggacatccagatgacccagaccaccagcagcctgagcgccagcctgggcgatagagtgaccatcagctgcagagccagccaggacatcagcaagtacctgaactggtatcagcagaaacccgacggcaccgtgaagctgctgatctaccacaccagcagactgcacagcggcgtgcccagcagattttctggcagcggctccggcaccgactacagcctgaccatctccaacctggaacaggaagatatcgctacctacttctgtcagcaaggcaacaccctgccctacaccttcggcggaggcaccaagctggaaatcacaggcggcggaggatctggcggaggcggaagtggcggagggggatctgaagtgaaactgcaggaaagcggccctggcctggtggccccatctcagtctctgagcgtgacctgtaccgtgtccggcgtgtccctgcctgactatggcgtgtcctggatcagacagccccccagaaagggcctggaatggctgggagtgatctggggcagcgagacaacctactacaacagcgccctgaagtcccggctgaccatcatcaaggacaactccaagagccaggtgttcctgaagatgaacagcctgcagaccgacgacaccgccatctactactgcgccaagcactactactacggcggcagctacgccatggactactggggccagggcacaagcgtgaccgtgtctagcacaaccacccctgcccctagacctccaaccccagcccctacaatcgccagccagcctctgtctctgaggcccgaggcttgtagaccagctgctggcggagccgtgcacaccagaggactggatttcgcctgcgacatctacatctgggcccctctggccggcacatgtggcgtgctgctgctgagcctcgtgatcaccctgtactgcggatccaagcggggcagaaagaaactgctgtacatctttaagcagcccttcatgcggcccgtgcagaccacccaggaagaggacggctgctcctgcagattccccgaggaagaagaaggcggctgcgagctgagatccggatctggaagtggctccctgagagtgaagtttagcagaagcgccgacgcccctgcctatcagcagggacagaaccagctgtataacgagctgaacctgggcaggcgggaagagtacgacgtgctggataagaggcggggcagggaccctgaaatgggcggcaaacccagacggaagaacccccaggaaggcctgtacaacgaactgcagaaagacaagatggccgaggcctacagcgagatcggaatgaagggcgagcggcggagaggcaagggacatgatggcctgtaccagggcctgtccaccgccaccaaggacacctatgacgccctgcacatgcaggccctgcctccaagaggcagcggatctggcagtggaagcgatagaagaggcggcagaatgctgaaacacaagcggcagagggacgacggggaaggcagaggcgaagtgggatctgccggcgatatgagagccgccaacctgtggcctagccccctgatgatcaagcggagcaagaagaactccctggccctgagcctgaccgccgaccagatggtgtctgccctgctggatgccgagccccccatcctgtacagcgagtacgaccccaccagacccttcagcgaggccagcatgatgggcctgctgaccaacctggccgaccgggaactggtgcacatgatcaactgggccaagcgggtgcccggcttcgtggatctgacactgcacgaccaggtgcacctgctggaatgcgcttggctggaaatcctgatgatcggcctcgtgtggcggagcatggaacaccctggcaagctgctgttcgcccccaacctgctgctggaccggaaccagggcaaatgcgtggaaggcatggtggaaatcttcgacatgctgctggccacctccagccggttccggatgatgaacctgcagggcgaagagttcgtgtgtctgaagtccatcatcctgctgaatagcggcgtgtacaccttcctgagcagcaccctgaaaagcctggaagaaaaggaccacatccaccgggtgctggacaagatcaccgacaccctgattcacctgatggccaaggccggactgaccctgcagcagcagcatcagagactggctcagctgctgctgatcctgtcccacatccggcacatgagcaacaagcggatggaacatctgtacagcatgaagtgcaagaacgtggtgcctctgttcgatctgctgctggaaatgctggacgcccacaggctgcacgccccaacatccggatctggctctggaagcggcagcatggtgtctaagggggaagaggacaacatggccatcatcaaagaattcatgcggttcaaggtgcacatggaaggctccgtgaatggccacgaattcgagatcgagggggagggcgagggcagaccttatgagggaacccagaccgccaagctgaaagtgaccaagggcggacccctgcctttcgcctgggatatcctgtctccccagtttatgtacggcagcaaggcctacgtgaagcaccccgccgacatccccgactacctgaagctgagcttccctgagggcttcaagtgggagagagtgatgaatttcgaggacggcggagtcgtgacagtgacccaggatagctctctgcaggacggcgagttcatctacaaagtgaagctgcggggcaccaacttccccagcgacggacccgtgatgcagaaaaagaccatgggctgggaggccagctccgagagaatgtacccagaggacggggccctgaagggggagatcaagcagcggctgaaactgaaggatggcggccactacgacgcagaagtgaaaaccacctacaaggccaagaaacctgtgcagctgcctggcgcctacaatgtgaacatcaagctggacattaccagccacaacgaggactacaccatcgtggaacagtacgagcgggccgagggcaggcattctacaggcggaatggatgaactgtataagtgcgtgaccgactag

SEQ ID NO: 33 - protein, 1060 aa, Artificial Sequence
  v.3 construct
MALPVTALLLPLALLLHAARPEQKLISEEDLDIQMTQTTSSLSASLGDRVTISCRASQDISKYLNWYQQKPDGTVKLLIYHTSRLHSGVPSRFSGSGSGTDYSLTISNLEQEDIATYFCQQGNTLPYTFGGGTKLEITGGGGSGGGGSGGGGSEVKLQESGPGLVAPSQSLSVTCTVSGVSLPDYGVSWIRQPPRKGLEWLGVIWGSETTYYNSALKSRLTIIKDNSKSQVFLKMNSLQTDDTAIYYCAKHYYYGGSYAMDYWGQGTSVTVSSTTTPAPRPPTPAPTIASQPLSLRPEACRPAAGGAVHTRGLDFACDIYIWAPLAGTCGVLLLSLVITLYCGSKRGRKKLLYIFKQPFMRPVQTTQEEDGCSCRFPEEEEGGCELRSGSGSGSLRVKFSRSADAPAYQQGQNQLYNELNLGRREEYDVLDKRRGRDPEMGGKPRRKNPQEGLYNELQKDKMAEAYSEIGMKGERRRGKGHDGLYQGLSTATKDTYDALHMQALPPRGSGSGSGSDRRGGRMLKHKRQRDDGEGRGEVGSAGDMRAANLWPSPLMIKRSKKNSLALSLTADQMVSALLDAEPPILYSEYDPTRPFSEASMMGLLTNLADRELVHMINWAKRVPGFVDLTLHDQVHLLECAWLEILMIGLVWRSMEHPGKLLFAPNLLLDRNQGKCVEGMVEIFDMLLATSSRFRMMNLQGEEFVCLKSIILLNSGVYTFLSSTLKSLEEKDHIHRVLDKITDTLIHLMAKAGLTLQQQHQRLAQLLLILSHIRHMSNKRMEHLYSMKCKNVVPLFDLLLEMLDAHRLHAPTSGSGSGSGSMVSKGEEDNMAIIKEFMRFKVHMEGSVNGHEFEIEGEGEGRPYEGTQTAKLKVTKGGPLPFAWDILSPQFMYGSKAYVKHPADIPDYLKLSFPEGFKWERVMNFEDGGVVTVTQDSSLQDGEFIYKVKLRGTNFPSDGPVMQKKTMGWEASSERMYPEDGALKGEIKQRLKLKDGGHYDAEVKTTYKAKKPVQLPGAYNVNIKLDITSHNEDYTIVEQYERAEGRHSTGGMDELYKCVTD

SEQ ID NO: 34 - DNA, 3206 bp, Artificial Sequence
  v.4 construct
atggctctgcctgtgacagctctgctgctgcctctggccctgctgctgcatgccgctagacctgagcagaagctgatctccgaagaggacctggacatccagatgacccagaccaccagcagcctgagcgccagcctgggcgatagagtgaccatcagctgcagagccagccaggacatcagcaagtacctgaactggtatcagcagaaacccgacggcaccgtgaagctgctgatctaccacaccagcagactgcacagcggcgtgcccagcagattttctggcagcggctccggcaccgactacagcctgaccatctccaacctggaacaggaagatatcgctacctacttctgtcagcaaggcaacaccctgccctacaccttcggcggaggcaccaagctggaaatcacaggcggcggaggatctggcggaggcggaagtggcggagggggatctgaagtgaaactgcaggaaagcggccctggcctggtggccccatctcagtctctgagcgtgacctgtaccgtgtccggcgtgtccctgcctgactatggcgtgtcctggatcagacagccccccagaaagggcctggaatggctgggagtgatctggggcagcgagacaacctactacaacagcgccctgaagtcccggctgaccatcatcaaggacaactccaagagccaggtgttcctgaagatgaacagcctgcagaccgacgacaccgccatctactactgcgccaagcactactactacggcggcagctacgccatggactactggggccagggcacaagcgtgaccgtgtctagcacaaccacccctgcccctagacctccaaccccagcccctacaatcgccagccagcctctgtctctgaggcccgaggcttgtagaccagctgctggcggagccgtgcacaccagaggactggatttcgcctgcgacatctacatctgggcccctctggccggcacatgtggcgtgctgctgctgagcctcgtgatcaccctgtactgcggatccggcagcggatctggcagtggaagcgatagaagaggcggcagaatgctgaaacacaagcggcagagggacgacggggaaggcagaggcgaagtgggatctgccggcgatatgagagccgccaacctgtggcctagccccctgatgatcaagcggagcaagaagaactccctggccctgagcctgaccgccgaccagatggtgtctgccctgctggatgccgagccccccatcctgtacagcgagtacgaccccaccagacccttcagcgaggccagcatgatgggcctgctgaccaacctggccgaccgggaactggtgcacatgatcaactgggccaagcgggtgcccggcttcgtggatctgacactgcacgaccaggtgcacctgctggaatgcgcttggctggaaatcctgatgatcggcctcgtgtggcggagcatggaacaccctggcaagctgctgttcgcccccaacctgctgctggaccggaaccagggcaaatgcgtggaaggcatggtggaaatcttcgacatgctgctggccacctccagccggttccggatgatgaacctgcagggcgaagagttcgtgtgtctgaagtccatcatcctgctgaatagcggcgtgtacaccttcctgagcagcaccctgaaaagcctggaagaaaaggaccacatccaccgggtgctggacaagatcaccgacaccctgattcacctgatggccaaggccggactgaccctgcagcagcagcatcagagactggctcagctgctgctgatcctgtcccacatccggcacatgagcaacaagcggatggaacatctgtacagcatgaagtgcaagaacgtggtgcctctgttcgatctgctgctggaaatgctggacgcccacaggctgcacgccccaacatccggatctggctctggaagcggcagcaagcggggcagaaagaaactgctgtacatctttaagcagcccttcatgcggcccgtgcagaccacccaggaagaggacggctgctcctgcagattccccgaggaagaagaaggcggctgcgagctgagatccggatctggaagtggctccctgagagtgaagtttagcagaagcgccgacgcccctgcctatcagcagggacagaaccagctgtataacgagctgaacctgggcaggcgggaagagtacgacgtgctggataagaggcggggcagggaccctgaaatgggcggcaaacccagacggaagaacccccaggaaggcctgtacaacgaactgcagaaagacaagatggccgaggcctacagcgagatcggaatgaagggcgagcggcggagaggcaagggacatgatggcctgtaccagggcctgtccaccgccaccaaggacacctatgacgccctgcacatgcaggccctgcctccaagaggaagtggatctgggagcggctctatggtgtctaagggggaagaggacaacatggccatcatcaaagaattcatgcggttcaaggtgcacatggaaggctccgtgaatggccacgaattcgagatcgagggggagggcgagggcagaccttatgagggaacccagaccgccaagctgaaagtgaccaagggcggacccctgcctttcgcctgggatatcctgtctccccagtttatgtacggcagcaaggcctacgtgaagcaccccgccgacatccccgactacctgaagctgagcttccctgagggcttcaagtgggagagagtgatgaatttcgaggacggcggagtcgtgacagtgacccaggatagctctctgcaggacggcgagttcatctacaaagtgaagctgcggggcaccaacttccccagcgacggacccgtgatgcagaaaaagaccatgggctgggaggccagctccgagagaatgtacccagaggacggggccctgaagggggagatcaagcagcggctgaaactgaaggatggcggccactacgacgcagaagtgaaaaccacctacaaggccaagaaacctgtgcagctgcctggcgcctacaatgtgaacatcaagctggacattaccagccacaacgaggactacaccatcgtggaacagtacgagcgggccgagggcaggcattctacaggcggaatggatgaactgtataagtgcgtgaccgacta

SEQ ID NO: 35 - protein, 1068 aa, Artificial Sequence
  v.4 construct
MALPVTALLLPLALLLHAARPEQKLISEEDLDIQMTQTTSSLSASLGDRVTISCRASQDISKYLNWYQQKPDGTVKLLIYHTSRLHSGVPSRFSGSGSGTDYSLTISNLEQEDIATYFCQQGNTLPYTFGGGTKLEITGGGGSGGGGSGGGGSEVKLQESGPGLVAPSQSLSVTCTVSGVSLPDYGVSWIRQPPRKGLEWLGVIWGSETTYYNSALKSRLTIIKDNSKSQVFLKMNSLQTDDTAIYYCAKHYYYGGSYAMDYWGQGTSVTVSSTTTPAPRPPTPAPTIASQPLSLRPEACRPAAGGAVHTRGLDFACDIYIWAPLAGTCGVLLLSLVITLYCGSGSGSGSGSDRRGGRMLKHKRQRDDGEGRGEVGSAGDMRAANLWPSPLMIKRSKKNSLALSLTADQMVSALLDAEPPILYSEYDPTRPFSEASMMGLLTNLADRELVHMINWAKRVPGFVDLTLHDQVHLLECAWLEILMIGLVWRSMEHPGKLLFAPNLLLDRNQGKCVEGMVEIFDMLLATSSRFRMMNLQGEEFVCLKSIILLNSGVYTFLSSTLKSLEEKDHIHRVLDKITDTLIHLMAKAGLTLQQQHQRLAQLLLILSHIRHMSNKRMEHLYSMKCKNVVPLFDLLLEMLDAHRLHAPTSGSGSGSGSKRGRKKLLYIFKQPFMRPVQTTQEEDGCSCRFPEEEEGGCELRSGSGSGSLRVKFSRSADAPAYQQGQNQLYNELNLGRREEYDVLDKRRGRDPEMGGKPRRKNPQEGLYNELQKDKMAEAYSEIGMKGERRRGKGHDGLYQGLSTATKDTYDALHMQALPPRGSGSGSGSMVSKGEEDNMAIIKEFMRFKVHMEGSVNGHEFEIEGEGEGRPYEGTQTAKLKVTKGGPLPFAWDILSPQFMYGSKAYVKHPADIPDYLKLSFPEGFKWERVMNFEDGGVVTVTQDSSLQDGEFIYKVKLRGTNFPSDGPVMQKKTMGWEASSERMYPEDGALKGEIKQRLKLKDGGHYDAEVKTTYKAKKPVQLPGAYNVNIKLDITSHNEDYTIVEQYERAEGRHSTGGMDELYKCVTD

SEQ ID NO: 36 - DNA, 2694 bp, Artificial Sequence
  v.5 construct
atggctctgcctgtgacagctctgctgctgcctctggccctgctgctgcatgccgctagacctgagcagaagctgatctccgaagaggacctggacatccagatgacccagaccaccagcagcctgagcgccagcctgggcgatagagtgaccatcagctgcagagccagccaggacatcagcaagtacctgaactggtatcagcagaaacccgacggcaccgtgaagctgctgatctaccacaccagcagactgcacagcggcgtgcccagcagattttctggcagcggctccggcaccgactacagcctgaccatctccaacctggaacaggaagatatcgctacctacttctgtcagcaaggcaacaccctgccctacaccttcggcggaggcaccaagctggaaatcacaggcggcggaggatctggcggaggcggaagtggcggagggggatctgaagtgaaactgcaggaaagcggccctggcctggtggccccatctcagtctctgagcgtgacctgtaccgtgtccggcgtgtccctgcctgactatggcgtgtcctggatcagacagccccccagaaagggcctggaatggctgggagtgatctggggcagcgagacaacctactacaacagcgccctgaagtcccggctgaccatcatcaaggacaactccaagagccaggtgttcctgaagatgaacagcctgcagaccgacgacaccgccatctactactgcgccaagcactactactacggcggcagctacgccatggactactggggccagggcacaagcgtgaccgtgtctagcacaaccacccctgcccctagacctccaaccccagcccctacaatcgccagccagcctctgtctctgaggcccgaggcttgtagaccagctgctggcggagccgtgcacaccagaggactggatttcgcctgcgacatctacatctgggcccctctggccggcacatgtggcgtgctgctgctgagcctcgtgatcaccctgtactgcggatccggcagcggatctggcagtggaagcgatagaagaggcggcagaatgctgaaacacaagcggcagagggacgacggggaaggcagaggcgaagtgggatctgccggcgatatgagagccgccaacctgtggcctagccccctgatgatcaagcggagcaagaagaactccctggccctgagcctgaccgccgaccagatggtgtctgccctgctggatgccgagccccccatcctgtacagcgagtacgaccccaccagacccttcagcgaggccagcatgatgggcctgctgaccaacctggccgaccgggaactggtgcacatgatcaactgggccaagcgggtgcccggcttcgtggatctgacactgcacgaccaggtgcacctgctggaatgcgcttggctggaaatcctgatgatcggcctcgtgtggcggagcatggaacaccctggcaagctgctgttcgcccccaacctgctgctggaccggaaccagggcaaatgcgtggaaggcatggtggaaatcttcgacatgctgctggccacctccagccggttccggatgatgaacctgcagggcgaagagttcgtgtgtctgaagtccatcatcctgctgaatagcggcgtgtacaccttcctgagcagcaccctgaaaagcctggaagaaaaggaccacatccaccgggtgctggacaagatcaccgacaccctgattcacctgatggccaaggccggactgaccctgcagcagcagcatcagagactggctcagctgctgctgatcctgtcccacatccggcacatgagcaacaagcggatggaacatctgtacagcatgaagtgcaagaacgtggtgcctctgttcgatctgctgctggaaatgctggacgcccacaggctgcacgccccaacatccggatctggctctggaagcggcagcatggtgtctaagggggaagaggacaacatggccatcatcaaagaattcatgcggttcaaggtgcacatggaaggctccgtgaatggccacgaattcgagatcgagggggagggcgagggcagaccttatgagggaacccagaccgccaagctgaaagtgaccaagggcggacccctgcctttcgcctgggatatcctgtctccccagtttatgtacggcagcaaggcctacgtgaagcaccccgccgacatccccgactacctgaagctgagcttccctgagggcttcaagtgggagagagtgatgaatttcgaggacggcggagtcgtgacagtgacccaggatagctctctgcaggacggcgagttcatctacaaagtgaagctgcggggcaccaacttccccagcgacggacccgtgatgcagaaaaagaccatgggctgggaggccagctccgagagaatgtacccagaggacggggccctgaagggggagatcaagcagcggctgaaactgaaggatggcggccactacgacgcagaagtgaaaaccacctacaaggccaagaaacctgtgcagctgcctggcgcctacaatgtgaacatcaagctggacattaccagccacaacgaggactacaccatcgtggaacagtacgagcgggccgagggcaggcattctacaggcggaatggatgaactgtataagtgcgtgaccgactag

SEQ ID NO: 37 - protein, 897 aa, Artificial Sequence
  v.5 construct
MALPVTALLLPLALLLHAARPEQKLISEEDLDIQMTQTTSSLSASLGDRVTISCRASQDISKYLNWYQQKPDGTVKLLIYHTSRLHSGVPSRFSGSGSGTDYSLTISNLEQEDIATYFCQQGNTLPYTFGGGTKLEITGGGGSGGGGSGGGGSEVKLQESGPGLVAPSQSLSVTCTVSGVSLPDYGVSWIRQPPRKGLEWLGVIWGSETTYYNSALKSRLTIIKDNSKSQVFLKMNSLQTDDTAIYYCAKHYYYGGSYAMDYWGQGTSVTVSSTTTPAPRPPTPAPTIASQPLSLRPEACRPAAGGAVHTRGLDFACDIYIWAPLAGTCGVLLLSLVITLYCGSGSGSGSGSDRRGGRMLKHKRQRDDGEGRGEVGSAGDMRAANLWPSPLMIKRSKKNSLALSLTADQMVSALLDAEPPILYSEYDPTRPFSEASMMGLLTNLADRELVHMINWAKRVPGFVDLTLHDQVHLLECAWLEILMIGLVWRSMEHPGKLLFAPNLLLDRNQGKCVEGMVEIFDMLLATSSRFRMMNLQGEEFVCLKSIILLNSGVYTFLSSTLKSLEEKDHIHRVLDKITDTLIHLMAKAGLTLQQQHQRLAQLLLILSHIRHMSNKRMEHLYSMKCKNVVPLFDLLLEMLDAHRLHAPTSGSGSGSGSMVSKGEEDNMAIIKEFMRFKVHMEGSVNGHEFEIEGEGEGRPYEGTQTAKLKVTKGGPLPFAWDILSPQFMYGSKAYVKHPADIPDYLKLSFPEGFKWERVMNFEDGGVVTVTQDSSLQDGEFIYKVKLRGTNFPSDGPVMQKKTMGWEASSERMYPEDGALKGEIKQRLKLKDGGHYDAEVKTTYKAKKPVQLPGAYNVNIKLDITSHNEDYTIVEQYERAEGRHSTGGMDELYKCVTD

SEQ ID NO: 38 - DNA, 2391 bp, Artificial Sequence
  ERa-LBD fusion protein with FLAG construct
atgatccacctgggacacatcctgtttttgctgctgctgccagtggctgccgccgattacaaagacgacgatgataaacagacaacaccaggcgagagatctagcctgcccgccttctaccctggcaccagcggctcttgttctggctgtggcagcctgtctctgcccatctatatttgggcacccctggctggaacctgcggagtgctgctgctgtctctcgtgattacactgtattgcaaaaggggccggaaaaagctgctgtatattttcaaacagccttttatgaggcctgtgcagacaacacaggaagaggacggctgtagctgtcggttccccgaagaggaagaggggggctgcgaactgggatcaggcagtggctctggcagcgatagaagaggcggcagaatgctgaaacacaagcggcagagggacgacggggaaggcagaggcgaagtgggatctgccggcgatatgagagccgccaacctgtggcctagccccctgatgatcaagcggagcaagaagaactccctggccctgagcctgaccgccgaccagatggtgtctgccctgctggatgccgagccccccatcctgtacagcgagtacgaccccaccagacccttcagcgaggccagcatgatgggcctgctgaccaacctggccgaccgggaactggtgcacatgatcaactgggccaagcgggtgcccggcttcgtggatctgacactgcacgaccaggtgcacctgctggaatgcgcttggctggaaatcctgatgatcggcctcgtgtggcggagcatggaacaccctggcaagctgctgttcgcccccaacctgctgctggaccggaaccagggcaaatgcgtggaaggcatggtggaaatcttcgacatgctgctggccacctccagccggttccggatgatgaacctgcagggcgaagagttcgtgtgtctgaagtccatcatcctgctgaatagcggcgtgtacaccttcctgagcagcaccctgaaaagcctggaagaaaaggaccacatccaccgggtgctggacaagatcaccgacaccctgattcacctgatggccaaggccggactgaccctgcagcagcagcatcagagactggctcagctgctgctgatcctgtcccacatccggcacatgagcaacaagcggatggaacatctgtacagcatgaagtgcaagaacgtggtgcctctgttcgatctgctgctggaaatgctggacgcccacaggctgcacgccccaacatccagatccggatctggaagtggctccctgagagtgaagtttagcagaagcgccgacgcccctgcctatcagcagggacagaaccagctgtataacgagctgaacctgggcaggcgggaagagtacgacgtgctggataagaggcggggcagggaccctgaaatgggcggcaaacccagacggaagaacccccaggaaggcctgtacaacgaactgcagaaagacaagatggccgaggcctacagcgagatcggaatgaagggcgagcggcggagaggcaagggacatgatggcctgtaccagggcctgtccaccgccaccaaggacacctatgacgccctgcacatgcaggccctgcctccaagaggaagtggatctgggagcggctctatggtgtctaagggggaagaggacaacatggccatcatcaaagaattcatgcggttcaaggtgcacatggaaggctccgtgaatggccacgaattcgagatcgagggggagggcgagggcagaccttatgagggaacccagaccgccaagctgaaagtgaccaagggcggacccctgcctttcgcctgggatatcctgtctccccagtttatgtacggcagcaaggcctacgtgaagcaccccgccgacatccccgactacctgaagctgagcttccctgagggcttcaagtgggagagagtgatgaatttcgaggacggcggagtcgtgacagtgacccaggatagctctctgcaggacggcgagttcatctacaaagtgaagctgcggggcaccaacttccccagcgacggacccgtgatgcagaaaaagaccatgggctgggaggccagctccgagagaatgtacccagaggacggggccctgaagggggagatcaagcagcggctgaaactgaaggatggcggccactacgacgcagaagtgaaaaccacctacaaggccaagaaacctgtgcagctgcctggcgcctacaatgtgaacatcaagctggacattaccagccacaacgaggactacaccatcgtggaacagtacgagcgggccgagggcaggcattctacaggcggaatggatgaactgtataagtgcgtgaccgactag

SEQ ID NO: 39 - protein, 796 aa, Artificial Sequence
  ERa-LBD fusion protein with FLAG construct
MIHLGHILFLLLLPVAAADYKDDDDKQTTPGERSSLPAFYPGTSGSCSGCGSLSLPIYIWAPLAGTCGVLLLSLVITLYCKRGRKKLLYIFKQPFMRPVQTTQEEDGCSCRFPEEEEGGCELGSGSGSGSDRRGGRMLKHKRQRDDGEGRGEVGSAGDMRAANLWPSPLMIKRSKKNSLALSLTADQMVSALLDAEPPILYSEYDPTRPFSEASMMGLLTNLADRELVHMINWAKRVPGFVDLTLHDQVHLLECAWLEILMIGLVWRSMEHPGKLLFAPNLLLDRNQGKCVEGMVEIFDMLLATSSRFRMMNLQGEEFVCLKSIILLNSGVYTFLSSTLKSLEEKDHIHRVLDKITDTLIHLMAKAGLTLQQQHQRLAQLLLILSHIRHMSNKRMEHLYSMKCKNVVPLFDLLLEMLDAHRLHAPTSRSGSGSGSLRVKFSRSADAPAYQQGQNQLYNELNLGRREEYDVLDKRRGRDPEMGGKPRRKNPQEGLYNELQKDKMAEAYSEIGMKGERRRGKGHDGLYQGLSTATKDTYDALHMQALPPRGSGSGSGSMVSKGEEDNMAIIKEFMRFKVHMEGSVNGHEFEIEGEGEGRPYEGTQTAKLKVTKGGPLPFAWDILSPQFMYGSKAYVKHPADIPDYLKLSFPEGFKWERVMNFEDGGVVTVTQDSSLQDGEFIYKVKLRGTNFPSDGPVMQKKTMGWEASSERMYPEDGALKGEIKQRLKLKDGGHYDAEVKTTYKAKKPVQLPGAYNVNIKLDITSHNEDYTIVEQYERAEGRHSTGGMDELYKCVTD

SEQ ID NO: 40 - protein, 18 aa, Homo sapiens
MIHLGHILFLLLLPVAAA

SEQ ID NO: 41 - protein, 8 aa, Artificial Sequence
  FLAG tag
DYKDDDDK

SEQ ID NO: 42 - protein, 30 aa, Homo sapiens
QTTPGERSSLPAFYPGTSGSCSGCGSLSLP

SEQ ID NO: 43 - protein, 24 aa, Homo sapiens
IYIWAPLAGTCGVLLLSLVITLYC

SEQ ID NO: 44 - protein, 42 aa, Homo sapiens
KRGRKKLLYIFKQPFMRPVQTTQEEDGCSCRFPEEEEGGCEL

SEQ ID NO: 45 - protein, 8 aa, Artificial Sequence
  Linker sequence
GSGSGSGS

SEQ ID NO: 46 - protein, 297 aa, Artificial Sequence; identical to SEQ ID NO: 28
  Modified ERa ligand binding domain

SEQ ID NO: 47 - protein, 8 aa, Artificial Sequence
  Linker sequence
RSGSGSGS

SEQ ID NO: 48 - protein, 113 aa, Homo sapiens
LRVKFSRSADAPAYQQGQNQLYNELNLGRREEYDVLDKRRGRDPEMGGKPRRKNPQEGLYNELQKDKMAEAYSEIGMKGERRRGKGHDGLYQGLSTATKDTYDALHMQALPPR

SEQ ID NO: 49 - protein, 8 aa, Artificial Sequence
  Linker sequence
GSGSGSGS

SEQ ID NO: 50 - protein, 240 aa, Artificial Sequence
  mCherry
MVSKGEEDNMAIIKEFMRFKVHMEGSVNGHEFEIEGEGEGRPYEGTQTAKLKVTKGGPLPFAWDILSPQFMYGSKAYVKHPADIPDYLKLSFPEGFKWERVMNFEDGGVVTVTQDSSLQDGEFIYKVKLRGTNFPSDGPVMQKKTMGWEASSERMYPEDGALKGEIKQRLKLKDGGHYDAEVKTTYKAKKPVQLPGAYNVNIKLDITSHNEDYTIVEQYERAEGRHSTGGMDELYKCVTD

SEQ ID NO: 51 - DNA, 2265 bp, Artificial Sequence
  PR ligand-binding domain construct
atgatccacctgggacacatcctgtttttgctgctgctgccagtggctgccgccgattacaaagacgacgatgataaacagacaacaccaggcgagagatctagcctgcccgccttctaccctggcaccagcggctcttgttctggctgtggcagcctgtctctgcccatctatatttgggcacccctggctggaacctgcggagtgctgctgctgtctctcgtgattacactgtattgcaaaaggggccggaaaaagctgctgtatattttcaaacagccttttatgaggcctgtgcagacaacacaggaagaggacggctgtagctgtcggttccccgaagaggaagaggggggctgcgaactgggatcaggcagtggctctggcagcgggcaagacattcagctcatacctcctttgataaatttgctgatgtctatagaaccagatgtcatatacgctggtcacgacaatacgaaaccggacacatcttcatctttgcttacctctctgaatcaactgggtgaacgacagctcctgagtgttgttaagtggtctaaaagcctcccgggcttcaggaatttgcacatagacgaccaaatcacgctcatccaatattcctggatgagtctcatggtctttggtctcggttggcgcagctataagcacgtctctggccagatgttgtatttcgcaccagacctgatcctgaacgaacagaggatgaaggaatcaagcttttactctctctgcttgactatgtggcaaatcccccaagaattcgtgaaacttcaagtttcccaagaagaattcctctgcatgaaagtccttcttttgctcaacacgattcccctggaaggcttgaggtctcaaacgcaattcgaggagatgcggagtagctatatacgcgaactcatcaaggccatcggtttgcggcaaaagggagtggtctctagtagccaacgattttaccagctgactaagctccttgacaaccttcacgatctcgtcaaacaactgcacctgtactgtcttaacacatttatacaatcacgggcactttctgtagagttcccagagatgatgtctgaggtcatcgcagcccaacttccgaaaattcttgcaggaatggtgaagccacttctgttccataagaaaagatccggatctggaagtggctccctgagagtgaagtttagcagaagcgccgacgcccctgcctatcagcagggacagaaccagctgtataacgagctgaacctgggcaggcgggaagagtacgacgtgctggataagaggcggggcagggaccctgaaatgggcggcaaacccagacggaagaacccccaggaaggcctgtacaacgaactgcagaaagacaagatggccgaggcctacagcgagatcggaatgaagggcgagcggcggagaggcaagggacatgatggcctgtaccagggcctgtccaccgccaccaaggacacctatgacgccctgcacatgcaggccctgcctccaagaggaagtggatctgggagcggctctatggtgtctaagggggaagaggacaacatggccatcatcaaagaattcatgcggttcaaggtgcacatggaaggctccgtgaatggccacgaattcgagatcgagggggagggcgagggcagaccttatgagggaacccagaccgccaagctgaaagtgaccaagggcggacccctgcctttcgcctgggatatcctgtctccccagtttatgtacggcagcaaggcctacgtgaagcaccccgccgacatccccgactacctgaagctgagcttccctgagggcttcaagtgggagagagtgatgaatttcgaggacggcggagtcgtgacagtgacccaggatagctctctgcaggacggcgagttcatctacaaagtgaagctgcggggcaccaacttccccagcgacggacccgtgatgcagaaaaagaccatgggctgggaggccagctccgagagaatgtacccagaggacggggccctgaagggggagatcaagcagcggctgaaactgaaggatggcggccactacgacgcagaagtgaaaaccacctacaaggccaagaaacctgtgcagctgcctggcgcctacaatgtgaacatcaagctggacattaccagccacaacgaggactacaccatcgtggaacagtacgagcgggccgagggcaggcattctacaggcggaatggatgaactgtataagtgcgtgaccgac

SEQ ID NO: 52 - protein, 755 aa, Artificial Sequence
  PR ligand-binding domain construct
MIHLGHILFLLLLPVAAADYKDDDDKQTTPGERSSLPAFYPGTSGSCSGCGSLSLPIYIWAPLAGTCGVLLLSLVITLYCKRGRKKLLYIFKQPFMRPVQTTQEEDGCSCRFPEEEEGGCELGSGSGSGSGQDIQLIPPLINLLMSIEPDVIYAGHDNTKPDTSSSLLTSLNQLGERQLLSVVKWSKSLPGFRNLHIDDQITLIQYSWMSLMVFGLGWRSYKHVSGQMLYFAPDLILNEQRMKESSFYSLCLTMWQIPQEFVKLQVSQEEFLCMKVLLLLNTIPLEGLRSQTQFEEMRSSYIRELIKAIGLRQKGVVSSSQRFYQLTKLLDNLHDLVKQLHLYCLNTFIQSRALSVEFPEMMSEVIAAQLPKILAGMVKPLLFHKKRSGSGSGSLRVKFSRSADAPAYQQGQNQLYNELNLGRREEYDVLDKRRGRDPEMGGKPRRKNPQEGLYNELQKDKMAEAYSEIGMKGERRRGKGHDGLYQGLSTATKDTYDALHMQALPPRGSGSGSGSMVSKGEEDNMAIIKEFMRFKVHMEGSVNGHEFEIEGEGEGRPYEGTQTAKLKVTKGGPLPFAWDILSPQFMYGSKAYVKHPADIPDYLKLSFPEGFKWERVMNFEDGGVVTVTQDSSLQDGEFIYKVKLRGTNFPSDGPVMQKKTMGWEASSERMYPEDGALKGEIKQRLKLKDGGHYDAEVKTTYKAKKPVQLPGAYNVNIKLDITSHNEDYTIVEQYERAEGRHSTGGMDELYKCVTD

SEQ ID NO: 53 - protein, 18 aa, Homo sapiens
MIHLGHILFLLLLPVAAA

SEQ ID NO: 54 - protein, 8 aa, Artificial Sequence
  FLAG tag
DYKDDDDK

SEQ ID NO: 55 - protein, 30 aa, Homo sapiens; identical to SEQ ID NO: 42

SEQ ID NO: 56 - protein, 24 aa, Homo sapiens
IYIWAPLAGTCGVLLLSLVITLYC

SEQ ID NO: 57 - protein, 42 aa, Homo sapiens; identical to SEQ ID NO: 44

SEQ ID NO: 58 - protein, 8 aa, Artificial Sequence
  Linker sequence
GSGSGSGS

SEQ ID NO: 59 - protein, 256 aa, Homo sapiens; identical to SEQ ID NO: 29

SEQ ID NO: 60 - protein, 8 aa, Artificial Sequence
  Linker sequence
RSGSGSGS

SEQ ID NO: 61 - protein, 113 aa, Homo sapiens; identical to SEQ ID NO: 48

SEQ ID NO: 62 - protein, 8 aa, Artificial Sequence
  Linker sequence
GSGSGSGS

SEQ ID NO: 63 - DNA, 54 bp, Artificial Sequence
  Dap10 signal
atgatccacctgggacacatcctgtttttgctgctgctgccagtggctgccgcc

SEQ ID NO: 64 - DNA, 24 bp, Artificial Sequence
  FLAG tag
gattacaaagacgacgatgataaa

SEQ ID NO: 65 - DNA, 90 bp, Artificial Sequence
  Dap10 extracellular domain
cagacaacaccaggcgagagatctagcctgcccgccttctaccctggcaccagcggctcttgttctggctgtggcagcctgtctctgccc

SEQ ID NO: 66 - DNA, 72 bp, Artificial Sequence
  CD8 transmembrane domain
atctatatttgggcacccctggctggaacctgcggagtgctgctgctgtctctcgtgattacactgtattgc

SEQ ID NO: 67 - DNA, 126 bp, Artificial Sequence
  4-1BB costimulatory domain
aaaaggggccggaaaaagctgctgtatattttcaaacagccttttatgaggcctgtgcagacaacacaggaagaggacggctgtagctgtcggttccccgaagaggaagaggggggctgcgaactg

SEQ ID NO: 68 - DNA, 24 bp, Artificial Sequence
  Linker sequence
ggatcaggcagtggctctggcagc

SEQ ID NO: 69 - DNA, 768 bp, Artificial Sequence
  Progesterone receptor ligand binding domain
gggcaagacattcagctcatacctcctttgataaatttgctgatgtctatagaaccagatgtcatatacgctggtcacgacaatacgaaaccggacacatcttcatctttgcttacctctctgaatcaactgggtgaacgacagctcctgagtgttgttaagtggtctaaaagcctcccgggcttcaggaatttgcacatagacgaccaaatcacgctcatccaatattcctggatgagtctcatggtctttggtctcggttggcgcagctataagcacgtctctggccagatgttgtatttcgcaccagacctgatcctgaacgaacagaggatgaaggaatcaagcttttactctctctgcttgactatgtggcaaatcccccaagaattcgtgaaacttcaagtttcccaagaagaattcctctgcatgaaagtccttcttttgctcaacacgattcccctggaaggcttgaggtctcaaacgcaattcgaggagatgcggagtagctatatacgcgaactcatcaaggccatcggtttgcggcaaaagggagtggtctctagtagccaacgattttaccagctgactaagctccttgacaaccttcacgatctcgtcaaacaactgcacctgtactgtcttaacacatttatacaatcacgggcactttctgtagagttcccagagatgatgtctgaggtcatcgcagcccaacttccgaaaattcttgcaggaatggtgaagccacttctgttccataagaaa

SEQ ID NO: 70 - DNA, 18 bp, Artificial Sequence
  Linker sequence
ggatctggaagtggctcc

SEQ ID NO: 71 - DNA, 339 bp, Artificial Sequence
  Sequence encoding CD3 zeta signaling domain
ctgagagtgaagtttagcagaagcgccgacgcccctgcctatcagcagggacagaaccagctgtataacgagctgaacctgggcaggcgggaagagtacgacgtgctggataagaggcggggcagggaccctgaaatgggcggcaaacccagacggaagaacccccaggaaggcctgtacaacgaactgcagaaagacaagatggccgaggcctacagcgagatcggaatgaagggcgagcggcggagaggcaagggacatgatggcctgtaccagggcctgtccaccgccaccaaggacacctatgacgccctgcacatgcaggccctgcctccaaga

SEQ ID NO: 72 - DNA, 24 bp, Artificial Sequence
  Linker sequence
ggaagtggatctgggagcggctct

SEQ ID NO: 73 - DNA, 720 bp, Artificial Sequence
  mCherry
atggtgtctaagggggaagaggacaacatggccatcatcaaagaattcatgcggttcaaggtgcacatggaaggctccgtgaatggccacgaattcgagatcgagggggagggcgagggcagaccttatgagggaacccagaccgccaagctgaaagtgaccaagggcggacccctgcctttcgcctgggatatcctgtctccccagtttatgtacggcagcaaggcctacgtgaagcaccccgccgacatccccgactacctgaagctgagcttccctgagggcttcaagtgggagagagtgatgaatttcgaggacggcggagtcgtgacagtgacccaggatagctctctgcaggacggcgagttcatctacaaagtgaagctgcggggcaccaacttccccagcgacggacccgtgatgcagaaaaagaccatgggctgggaggccagctccgagagaatgtacccagaggacggggccctgaagggggagatcaagcagcggctgaaactgaaggatggcggccactacgacgcagaagtgaaaaccacctacaaggccaagaaacctgtgcagctgcctggcgcctacaatgtgaacatcaagctggacattaccagccacaacgaggactacaccatcgtggaacagtacgagcgggccgagggcaggcattctacaggcggaatggatgaactgtataagtgcgtgaccgac

SEQ ID NO: 74 - protein, 480 aa, Homo sapiens
MERDEPPPSGGGGGGGSAGFLEPPAALPPPPRNGFCQDELAELDPGTISVSDDRAEQRTCLICGDRATGLHYGIISCEGCKGFFKRSICNKRVYRCSRDKNCVMSRKQRNRCQYCRLLKCLQMGMNRKAIREDGMPGGRNKSIGPVQISEEEIERIMSGQEFEEEANHWSNHGDSDHSSPGNRASESNQPSPGSTLSSSRSVELNGFMAFREQYMGMSVPPHYQYIPHLFSYSGHSPLLPQQARSLDPQSYSLIHQLLSAEDLEPLGTPMLIEDGYAVTQAELFALLCRLADELLFRQIAWIKKLPFFCELSIKDYTCLLSSTWQELILLSSLTVYSKQIFGELADVTAKYSPSDEELHRFSDEGMEVIERLIYLYHKFHQLKVSNEEYACMKAINFLNQDIRGLTSASQLEQLNKRYWYICQDFTEYKYTHQPNRFPDLMMCLPEIRYIAGKMVNVPLEQLPLLFKVVLHSCKTSVGKE

SEQ ID NO: 75 - protein, 505 aa, Homo sapiens
MGETLGDSPIDPESDSFTDTLSANISQEMTMVDTEMPFWPTNFGISSVDLSVMEDHSHSFDIKPFTTVDFSSISTPHYEDIPFTRTDPVVADYKYDLKLQEYQSAIKVEPASPPYYSEKTQLYNKPHEEPSNSLMAIECRVCGDKASGFHYGVHACEGCKGFFRRTIRLKLIYDRCDLNCRIHKKSRNKCQYCRFQKCLAVGMSHNAIRFGRMPQAEKEKLLAEISSDIDQLNPESADLRALAKHLYDSYIKSFPLTKAKARAILTGKTTDKSPFVIYDMNSLMMGEDKIKFKHITPLQEQSKEVAIRIFQGCQFRSVEAVQEITEYAKSIPGFVNLDLNDQVTLLKYGVHEIIYTMLASLMNKDGVLISEGQGFMTREFLKSLRKPFGDFMEPKFEFAVKFNALELDDSDLAIFIAVIILSGDRPGLLNVKPIEDIQDNLLQALELQLKLNHPESSQLFAKLLQKMTDLRQIVTEHVQLLQVIKKTETDMSLHPLLQEIYKDLY

SEQ ID NO: 76 - protein, 777 aa, Homo sapiens
MDSKESLTPGREENPSSVLAQERGDVMDFYKTLRGGATVKVSASSPSLAVASQSDSKQRRLLVDFPKGSVSNAQQPDLSKAVSLSMGLYMGETETKVMGNDLGFPQQGQISLSSGETDLKLLEESIANLNRSTSVPENPKSSASTAVSAAPTEKEFPKTHSDVSSEQQHLKGQTGTNGGNVKLYTTDQSTFDILQDLEFSSGSPGKETNESPWRSDLLIDENCLLSPLAGEDDSFLLEGNSNEDCKPLILPDTKPKIKDNGDLVLSSPSNVTLPQVKTEKEDFIELCTPGVIKQEKLGTVYCQASFPGANIIGNKMSAISVHGVSTSGGQMYHYDMNTASLSQQQDQKPIFNVIPPIPVGSENWNRCQGSGDDNLTSLGTLNFPGRTVFSNGYSSPSMRPDVSSPPSSSSTATTGPPPKLCLVCSDEASGCHYGVLTCGSCKVFFKRAVEGQHNYLCAGRNDCIIDKIRRKNCPACRYRKCLQAGMNLEARKTKKKIKGIQQATTGVSQETSENPGNKTIVPATLPQLTPTLVSLLEVIEPEVLYAGYDSSVPDSTWRIMTTLNMLGGRQVIAAVKWAKAIPGFRNLHLDDQMTLLQYSWMFLMAFALGWRSYRQSSANLLCFAPDLIINEQRMTLPCMYDQCKHMLYVSSELHRLQVSYEEYLCMKTLLLLSSVPKDGLKSQELFDEIRMTYIKELGKAIVKREGNSSQNWQRFYQLTKLLDSMHEVVENLLNYCFQTFLDKTMSIEFPEMLAEIITNQIPKYSNGNIKKLLFHQK

SEQ ID NO: 77 - protein, 490 aa, Homo sapiens
MEQKPSKVECGSDPEENSARSPDGKRKRKNGQCSLKTSMSGYIPSYLDKDEQCVVCGDKATGYHYRCITCEGCKGFFRRTIQKNLHPTYSCKYDSCCVIDKITRNQCQLCRFKKCIAVGMAMDLVLDDSKRVAKRKLIEQNRERRRKEEMIRSLQQRPEPTPEEWDLIHIATEAHRSTNAQGSHWKQRRKFLPDDIGQSPIVSMPDGDKVDLEAFSEFTKIITPAITRVVDFAKKLPMFSELPCEDQIILLKGCCMEIMSLRAAVRYDPESDTLTLSGEMAVKREQLKNGGLGVVSDAIFELGKSLSAFNLDDTEVALLQAVLLMSTDRSGLLCVDKIEKSQEAYLLAFEHYVNHRKHNIPHFWPKLLMKEREVQSSILYKGAAAEGRPGGSLGVHPEGQQLLGMHVVQGPQVRQLEQQLGEAGSLQGPVLQHQSPKSPQQRLLELLHRSGILHARAVCGEDDSSEADSPSSSEEEPEVCEDLAGNAASP

SEQ ID NO: 78 - protein, 924 aa, Homo sapiens
METKGYHSLPEGLDMERRWGQVSQAVERSSLGPTERTDENNYMEIVNVSCVSGAIPNNSTQGSSKEKQELLPCLQQDNNRPGILTSDIKTELESKELSATVAESMGLYMDSVRDADYSYEQQNQQGSMSPAKIYQNVEQLVKFYKGNGHRPSTLSCVNTPLRSFMSDSGSSVNGGVMRAIVKSPIMCHEKSPSVCSPLNMTSSVCSPAGINSVSSTTASFGSFPVHSPITQGTPLTCSPNAENRGSRSHSPAHASNVGSPLSSPLSSMKSSISSPPSHCSVKSPVSSPNNVTLRSSVSSPANINNSRCSVSSPSNTNNRSTLSSPAASTVGSICSPVNNAFSYTASGTSAGSSTLRDVVPSPDTQEKGAQEVPFPKTEEVESAISNGVTGQLNIVQYIKPEPDGAFSSSCLGGNSKINSDSSFSVPIKQESTKHSCSGTSFKGNPTVNPFPFMDGSYFSFMDDKDYYSLSGILGPPVPGFDGNCEGSGFPVGIKQEPDDGSYYPEASIPSSAIVGVNSGGQSFHYRIGAQGTISLSRSARDQSFQHLSSFPPVNTLVESWKSHGDLSSRRSDGYPVLEYIPENVSSSTLRSVSTGSSRPSKICLVCGDEASGCHYGVVTCGSCKVFFKRAVEGQHNYLCAGRNDCIIDKIRRKNCPACRLQKCLQAGMNLGARKSKKLGKLKGIHEEQPQQQQPPPPPPPPQSPEEGTTYIAPAKEPSVNTALVPQLSTISRALTPSPVMVLENIEPEIVYAGYDSSKPDTAENLLSTLNRLAGKQMIQVVKWAKVLPGFKNLPLEDQITLIQYSWMCLSSFALSWRSYKHTNSQFLYFAPDLVFNEEKMKELRKMVTKCPNNSGQSWQRFYQLTKLLDSMHDLVSDLLEFCFYTFRESHALKVEFPAMLVEIISDQLPKVESGNAKPLYFHRK

SEQ ID NO: 79 - protein, 427 aa, Homo sapiens
MEAMAASTSLPDPGDFDRNVPRICGVCGDRATGFHFNAMTCEGCKGFFRRSMKRKALFTCPFNGDCRITKDNRRHCQACRLKRCVDIGMMKEFILTDEEVQRKREMILKRKEEEALKDSLRPKLSEEQQRIIAILLDAHHKTYDPTYSDFCQFRPPVRVNDGGGSHPSRPNSRHTPSFSGDSSSSCSDHCITSSDMMDSSSFSNLDLSEEDSDDPSVTLELSQLSMLPHLADLVSYSIQKVIGFAKMIPGFRDLTSEDQIVLLKSSAIEVIMLRSNESFTMDDMSWTCGNQDYKYRVSDVTKAGHSLELIEPLIKFQVGLKKLNLHEEEHVLLMAICIVSPDRPGVQDAALIEAIQDRLSNTLQTYIRCRHPPPGSHLLYAKMIQKLADLRSLNEEHSKQYRCLSFQPECSMKLTPLVLEVFGNEIS

SEQ ID NO: 80 - protein, 468 aa, Hom sapiens
MVDTESPLCPLSPLEAGDLESPLSEEFLQEMGNIQEISQSIGEDSSGSFGFTEYQYLGSCPGSDGSVITDTLSPASSPSSVTYPVVPGSVDESPSGALNIECRICGDKASGYHYGVHACEGCKGFFRRTIRLKLVYDKCDRSCKIQKKNRNKCQYCRFHKCLSVGMSHNAIRFGRMPRSEKAKLKAEILTCEHDIEDSETADLKSLAKRIYEAYLKNFNMNKVKARVILSGKASNNPPFVIHDMETLCMAEKTLVAKLVANGIQNKEAEVRIFHCCQCTSVETVTELTEFAKAIPGFANLDLNDQVTLLKYGVYEAIFAMLSSVMNKDGMLVAYGNGFITREFLKSLRKPFCDIMEPKFDFAMKFNALELDDSDISLFVAAIICCGDRPGLLNVGHIEKMQEGIVHVLRLHLQSNHPDDIFLFPKLLQKMADLRQLVTEHAQLVQIIKKTESDAALHPLLQEIYRDMY

SEQ ID NO: 81 - protein, 441 aa, Homo sapiens
MEQPQEEAPEVREEEEKEEVAEAEGAPELNGGPQHALPSSSYTDLSRSSSPPSLLDQLQMGCDGASCGSLNMECRVCGDKASGFHYGVHACEGCKGFFRRTIRMKLEYEKCERSCKIQKKNRNKCQYCRFQKCLALGMSHNAIRFGRMPEAEKRKLVAGLTANEGSQYNPQVADLKAFSKHIYNAYLKNFNMTKKKARSILTGKASHTAPFVIHDIETLWQAEKGLVWKQLVNGLPPYKEISVHVFYRCQCTTVETVRELTEFAKSIPSFSSLFLNDQVTLLKYGVHEAIFAMLASIVNKDGLLVANGSGFVTREFLRSLRKPFSDIIEPKFEFAVKFNALELDDSDLALFIAAIILCGDRPGLMNVPRVEAIQDTILRALEFHLQANHPDAQYLFPKLLQKMADLRQLVTEHAQMMQRIKKTETETSLHPLLQEIYKDMY

SEQ ID NO: 82 - protein, 434 aa, Homo sapiens
MEVRPKESWNHADFVHCEDTESVPGKPSVNADEEVGGPQICRVCGDKATGYHFNVMTCEGCKGFFRRAMKRNARLRCPFRKGACEITRKTRRQCQACRLRKCLESGMKKEMIMSDEAVEERRALIKRKKSERTGTQPLGVQGLTEEQRMMIRELMDAQMKTFDTTFSHFKNFRLPGVLSSGCELPESLQAPSREEAAKWSQVRKDLCSLKVSLQLRGEDGSVWNYKPPADSGGKEIFSLLPHMADMSTYMFKGIISFAKVISYFRDLPIEDQISLLKGAAFELCQLRFNTVFNAETGTWECGRLSYCLEDTAGGFQQLLLEPMLKFHYMLKKLQLHEEEYVLMQAISLFSPDRPGVLQHRVVDQLQEQFAITLKSYIECNRPQPAHRFLFLKIMAMLTELRSINAQHTQRLLRIQDIHPFATPLMQELFGITGS

SEQ ID NO: 83 - protein, 257 aa, Homo sapiens
GSHMSQGSGEGEGVQLTAAQELMIQQLVAAQLQCNKRSFSDQPKVTPWPLGADPQSRDARQQRFAHFTELAIISVQEIVDFAKQVPGFLQLGREDQIALLKASTIEIMLLETARRYNHETECITFLKDFTYSKDDFHRAGLQVEFINPIFEFSRAMRRLGLDDAEYALLIAINIFSADRPNVQEPGRVEALQQPYVEALLSYTRIKRPQDQLRFPRMLMKLVSLRTLSSVHSEQVFALRLQDKKLPPLLSEIWDVHE

SEQ ID NO: 84 - protein, 472 aa, Homo sapiens
MGSKMNLIEHSHLPTTDEFSFSENLFGVLTEQVAGPLGQNLEVEPYSQYSNVQFPQVQPQISSSSYYSNLGFYPQQPEEWYSPGIYELRRMPAETLYQGETEVAEMPVTKKPRMGASAGRIKGDELCVVCGDRASGYHYNALTCEGCKGFFRRSITKNAVYKCKNGGNCVMDMYMRRKCQECRLRKCKEMGMLAECLLTEIQCKSKRLRKNVKQHADQTVNEDSEGRDLRQVTSTTKSCREKTELTPDQQTLLHFIMDSYNKQRMPQEITNKILKEEFSAEENFLILTEMATNHVQVLVEFTKKLPGFQTLDHEDQIALLKGSAVEAMFLRSAEIFNKKLPSGHSDLLEERIRNSGISDEYITPMFSFYKSIGELKMTQEEYALLTAIVILSPDRQYIKDREAVEKLQEPLLDVLQKLCKIHQPENPQHFACLLGRLTELRTFNHHHAEMLMSWRVNDHKFTPLLCEIWDVQ

SEQ ID NO: 85 - protein, 468 aa, Homo sapiens
MMYFVIAAMKAQIEIIPCKICGDKSSGIHYGVITCEGCKGFFRRSQQSNATYSCPRQKNCLIDRTSRNRCQHCRLQKCLAVGMSRDAVKFGRMSKKQRDSLYAEVQKHRMQQQQRDHQQQPGEAEPLTPTYNISANGLTELHDDLSNYIDGHTPEGSKADSAVSSFYLDIQPSPDQSGLDINGIKPEPICDYTPASGFFPYCSFTNGETSPTVSMAELEHLAQNISKSHLETCQYLREELQQITWQTFLQEEIENYQNKQREVMWQLCAIKITEAIQYVVEFAKRIDGFMELCQNDQIVLLKAGSLEVVFIRMCRAFDSQNNTVYFDGKYASPDVFKSLGCEDFISFVFEFGKSLCSMHLTEDEIALFSAFVLMSADRSWLQEKVKIEKLQQKIQLALQHVLQKNHREDGILTKLICKVSTLRALCGRHTEKLMAFKAIYPDIVRLHFPPLYKELFTSEFEPAMQIDG

SEQ ID NO: 86 - protein, 518 aa, Homo sapiens
MDRAPQRQHRASRELLAAKKTHTSQIEVIPCKICGDKSSGIHYGVITCEGCKGFFRRSQRCNAAYSCTRQQNCPIDRTSRNRCQHCRLQKCLALGMSRDAVKFGRMSKKQRDSLHAEVQKQLQQRQQQQQEPVVKTPPAGAQGADTLTYTLGLPDGQLPLGSSPDLPEASACPPGLLKASGSGPSYSNNLAKAGLNGASCHLEYSPERGKAEGRESFYSTGSQLTPDRCGLRFEEHRHPGLGELGQGPDSYGSPSFRSTPEAPYASLTEIEHLVQSVCKSYRETCQLRLEDLLRQRSNIFSREEVTGYQRKSMWEMWERCAHHLTEAIQYVVEFAKRLSGFMELCQNDQIVLLKAGAMEVVLVRMCRAYNADNRTVFFEGKYGGMELFRALGCSELISSIFDFSHSLSALHFSEDEIALYTALVLINAHRPGLQEKRKVEQLQYNLELAFHHHLCKTHRQSILAKLPPKGKLRSLCSQHVERLQIFQHLHPIVVQAAFPPLYKELFSTETESPVGLSK

SEQ ID NO: 87 - protein, 431 aa, Homo sapiens [sequence omitted]

SEQ ID NO: 88 - protein, 599 aa, Mus musculus
MTMTLHTKASGMALLHQIQGNELEPLNRPQLKMPMERALGEVYVDNSKPTVFNYPEGAAYEFNAAAAAAAAASAPVYGQSGIAYGPGSEAAAFSANSLGAFPQLNSVSPSPLMLLHPPPQLSPFLHPHGQQVPYYLENEPSAYAVRDTGPPAFYRSNSDNRRQNGRERLSSSNEKGNMIMESAKETRYCAVCNDYASGYHYGVWSCEGCKAFFKRSIQGHNDYMCPATNQCTIDKNRRKSCQACRLRKCYEVGMMKGGIRKDRRGGRMLKHKRQRDDLEGRNEMGASGDMRAANLWPSPLVIKHTKKNSPALSLTADQMVSALLDAEPPMIYSEYDPSRPFSEASMMGLLTNLADRELVHMINWAKRVPGFGDLNLHDQVHLLECAWLEILMIGLVWRSMEHPGKLLFAPNLLLDRNQGKCVEGMVEIFDMLLATSSRFRMMNLQGEEFVCLKSIILLNSGVYTFLSSTLKSLEEKDHIHRVLDKITDTLIHLMAKAGLTLQQQHRRLAQLLLILSHIRHMSNKGMEHLYNMKCKNVVPLYDLLLEMLDAHRLHAPASRMGVPPEEPSQTQLATTSSTSAHSLQTYYIPPEAEGFPNTI

SEQ ID NO: 89 - protein, 600 aa, Rattus rattus
MTMTLHTKASGMALLHQIQGNELEPLNRPQLKMPMERALGEVYVDNSKPAVFNYPEGAAYEFNAAAAAAAAGASAPVYGQSSITYGPGSEAAAFGANSLGAFPQLNSVSPSPLMLLHPPPHVSPFLHPHGHQVPYYLENEPSAYAVRDTGPPAFYRSNSDNRRQNGRERLSSSSEKGNMIMESAKETRYCAVCNDYASGYHYGVWSCEGCKAFFKRSIQGHNDYMCPATNQCTIDKNRRKSCQACRLRKCYEVGMMKGGIRKDRRGGRMLKHKRQRDDLEGRNEMGTSGDMRAANLWPSPLVIKHTKKNSPALSLTADQMVSALLDAEPPLIYSEYDPSRPFSEASMMGLLTNLADRELVHMINWAKRVPGFGDLNLHDQVHLLECAWLEILMIGLVWRSMEHPGKLLFAPNLLLDRNQGKCVEGMVEIFDMLLATSSRFRMMNLQGEEFVCLKSIILLNSGVYTFLSSTLKSLEEKDHIHRVLDKINDTLIHLMAKAGLTLQQQHRRLAQLLLILSHIRHMSNKGMEHLYNMKCKNVVPLYDLLLEMLDAHRLHAPASRMGVPPEEPSQSQLTTTSSTSAHSLQTYYIPPEAEGFPNTI

SEQ ID NO: 90 - protein, 595 aa, Papio Anubis
MTMTLHTKASGMALLHQIQGNELEPLNRPQLKIPLERPLGEVYVDSSKPAVYSYPEGAAYEFNAAAAANAQVYGQTGLPYGPGSEAAAFGSNGLGGFPPLNSVSPSPLMLLHPPPQLSPFLQPHGQQVPYYLENEPSGYTVREAGPPAFYRPNSDNRRQGGRERLASTNDKGSMAMESAKETRYCAVCNDYASGYHYGVWSCEGCKAFFKRSIQGHNDYMCPATNQCTIDKNRRKSCQACRLRKCYEVGMMKGGIRKDRRGGRMLKHKRQRDDGEGRGEVGSAGDMRAANLWPSPLMIKHSKKNSPALSLTADQMVSALLDAEPPILYSEYDPTRPFSEASMMGLLTNLADRELVHMINWAKRVPGFVDLTLHDQVHLLECAWLEILMIGLVWRSMEHPGKLLFAPNLLLDRNQGKCVEGMVEIFDMLLATSSRFRMMNLQGEEFVCLKSIILLNSGVYTFLSSTLKSLEEKDHIHRVLDKITDTLIHLMAKAGLTLQQQHRRLAQLLLILSHIRHMSNKGMEHLYSMKCKNVVPLYDLLLEMLDAHRLHAPTSRGGAPMEETDQSHLATAGSTSSHSLQKYYITGDAEGFPATV

SEQ ID NO: 91 - protein, 866 aa, Mus musculus
MTELQAKDPQVLHTSGASPSPPHIGSPLLARLDSGPFQGSQHSDVSSVVSPIPISLDGLLFPRSCRGPELPDGKTGDQQSLSDVEGAFSGVEATHREGGRNSRAPEKDSRLLDSVLDSLLTPSGTEQSHASPPACEAITSWCLFGPELPEDPRSVPATKGLLSPLMSRPEIKAGDSSGTGAGQKVLPKGLSPPRQLLLPTSGSAHWPGAGVKPSPQPAAGEVEEDSGLETEGSAAPLLKSKPRALEGTGSGGGVAANAASAAPGGVTLVPKEDSRFSAPRVSLEQDSPIAPGRSPLATTVVDFIHVPILPLNHALLAARTRQLLEGDSYDGGATAQGPFAPPRGSPSAPSPPVPCGDFPDCTYPLEGDPKEDVFPLYGDFQTPGLKIKEEEEGADAAVRSPRPYLSAGASSSTFPDFPLAPAPQRAPSSRPGEAAVAGGPSSAAVSPASSSGSALECILYKAEGAPPTQGSFAPLPCKPPAAGSCLLPRDSLPAAPATAAAPAIYQPLGLNGLPQLGYQAAVLKDSLPQVYPPYLNYLRPDSEASQSPQYGFDSLPQKICLICGDEASGCHYGVLTCGSCKVFFKRAMEGQHNYLCAGRNDCIVDKIRRKNCPACRLRKCCQAGMVLGGRKFKKFNKVRVMRTLDGVALPQSVGLPNESQALGQRITFSPNQEIQLVPPLINLLMSIEPDVVYAGHDNTKPDTSSSLLTSLNQLGERQLLRMKELSFYSLCLTMWQIPQEFVKLQVTHEEFLCMKVLLLLNTIPLEGLRSQSQFEEMRSSYIRELIKAIGLRQKGVVPSSQRFYQLTKLLDSLHDLVKQLHLYCLNTFIQSRTLAVEFPEMMSEVIAAQLPKILAGMVKPLLFHKK

SEQ ID NO: 92 - protein, 923 aa, Rattus rattus
MTELQAKDPRTLHTSGAAPSPTHVGSPLLARLDPDPFQGSQHSDASSVVSPIPISLDRLLFSRSCQAQELPDEKTQNQQSLSDVEGAFSGVEASRRRSRNPRAPEKDSRLLDSVLDTLLAPSGPEQSQTSPPACEAITSWCLFGPELPEDPRSVPATKGLLSPLMSRPESKAGDSSGTGAGQKVLPKAVSPPRQLLLPTSGSAHWPGAGVKPSQQPATVEVEEDGGLETEGSAGPLLKSKPRALEGMCSGGGVTANAPGAAPGGVTLVPKEDSRFSAPRVSLEQDAPVAPGRSPLATTVVDFIHVPILPLNHALLAARTRQLLEGDSYDGGAAAQVPFAPPRGSPSAPSPPVPCGDFPDCTYPPEGDPKEDGFPVYGEFQPPGLKIKEEEEGTEAASRSPRPYLLAGASAATFPDFPLPPRPPRAPPSRPGEAAVAAPSAAVSPVSSSGSALECILYKAEGAPPTQGSFAPLPCKPPAASSCLLPRDSLPAAPTSSAAPAIYPPLGLNGLPQLGYQAAVLKDSLPQVYPPYLNYLRPDSEASQSPQYGFDSLPQKICLICGDEASGCHYGVLTCGSCKVFFKRAMEGQHNYLCAGRNDCIVDKIRRKNCPACRLRKCCQAGMVLGGRKFKKFNKVRVMRALDGVALPQSVAFPNESQTLGQRITFSPNQEIQLVPPLINLLMSIEPDVVYAGHDNTKPDTSSSLLTSLNQLGERQLLSVVKWSKSLPGFRNLHIDDQITLIQYSWMSLMVFGLGWRSYKHVSGQMLYFAPDLILNEQRMKELSFYSLCLTMWQIPQEFVKLQVTHEEFLCMKVLLLLNTIPLEGLRSQSQFEEMRSSYIRELIKAIGLRQKGVVPSSQRFYQLTKLLDSLHDLVKQLHLYCLNTFIQSRALAVEFPEMMSEVIAAQLPKILAGMVKPLLFHKK

SEQ ID NO: 93 - protein, 933 aa, Papio anubis
MTELKAKGPRAPHVAGGPPSPEVGSPLLCRPAAGPFQGSQTSDTLPEVSAIPISLDGLLFPRPCQGQDPLDEKTQDQQSLSDVEGAYSRAEATRGTGGSSSRPPEKDSGLLHSVLDTLLAPSGPGQSQPSPPACEVTSSWCLFGPELPEDPPAAPATQGVLSPLMSRSGCKAGDSSGTAAAHKVLPRGLSPSRQLLLPASGSPHWSGAPVKPSPQPAAVEVEEEDGSESEESAGPLLKGKPRALGGAAAGGGAAAVPPGAAAGGVALVPKEDSRFSAPRVALVEQDAPMAPGRSPLATTTMDFTHVPILPLSHALLAARTRQLLEEESYDGGAGAASAFAPPRSSPSASSTPVAVGDFPDCAYPPDADPKDDAYPLYGDFQPPALKIKEEEEGAEVSARSPRSYLVAGANPAAFPDFPLGPPPPLPPRAPPSRPGEAAVTAAPAGASVSSASSSGSTLECILYKAEGAPPQQGPFAPPPCKAPGAGGCLLPRDGLPSTSASAAAAGAAPALYPALGLNGLPQLGYQAAVLKEGLQQVYPPYLNYLRPDSEASQSPQYSFESLPQKICLICGDEASGCHYGVLTCGSCKVFFKRAMEGQHNYLCAGRNDCIVDKIRRKNCPACRLRKCCQAGMVLGGRKFKKFNKVRVMRALDAVALPQPVGIPNESQALSQRFTFPPGQDIQLIPPLINLLVSIEPDVIYAGHDNSKPDTSSSLLTSLNQLGERQLLSVVKWSKLLPGFRNLHIDDQITLIQYSWMSLMVFGLGWRSYKHVSGQMLYFAPDLILNEQRMKESSFYSLCLTMWQIPQEFVKLQVSQEEFLCMKVLLLLNTIPLEGLRSQTQFEEMRSSYIRELIKAIGLRQKGVVSSSQRFYQLTKLLDNLHDLVKQLHLYCLNTFIQSRALSVEFPEMMSEVIAAQLPKILAGMVKPLLFHKK

SEQ ID NO: 94 - protein, 899 aa, Mus musculus
MEVQLGLGRVYPRPPSKTYRGAFQNLFQSVREAIQNPGPRHPEAANIAPPGACLQQRQETSPRRRRRQQHTEDGSPQAHIRGPTGYLALEEEQQPSQQQAASEGHPESSCLPEPGAATAPGKGLPQQPPAPPDQDDSAAPSTLSLLGPTFPGLSSCSADIKDILNEAGTMQLLQQQQQQQQHQQQHQQHQQQQEVISEGSSARAREATGAPSSSKDSYLGGNSTISDSAKELCKAVSVSMGLGVEALEHLSPGEQLRGDCMYASLLGGPPAVRPTPCAPLPECKGLPLDEGPGKSTEETAEYSSFKGGYAKGLEGESLGCSGSSEAGSSGTLEIPSSLSLYKSGALDEAAAYQNRDYYNFPLALSGPPHPPPPTHPHARIKLENPLDYGSAWAAAAAQCRYGDLGSLHGGSVAGPSTGSPPATTSSSWHTLFTAEEGQLYGPGGGGGSSSPSDAGPVAPYGYTRPPQGLTSQESDYSASEVWYPGGVVNRVPYPSPNCVKSEMGPWMENYSGPYGDMRLDSTRDHVLPIDYYFPPQKTCLICGDEASGCHYGALTCGSCKVFFKRAAEGKQKYLCASRNDCTIDKFRRKNCPSCRLRKCYEAGMTLGARKLKKLGNLKLQEEGENSNAGSPTEDPSQKMTVSHIEGYECQPIFLNVLEAIEPGVVCAGHDNNQPDSFAALLSSLNELGERQLVHVVKWAKALPGFRNLHVDDQMAVIQYSWMGLMVFAMGWRSFTNVNSRMLYFAPDLVFNEYRMHKSRMYSQCVRMRHLSQEFGWLQITPQEFLCMKALLLFSIIPVDGLKNQKFFDELRMNYIKELDRIIACKRKNPTSCSRRFYQLTKLLDSVQPIARELHQFTFDLLIKSHMVSVDFPEMMAEIISVQVPKILSGKVKPIYFHTQ

SEQ ID NO: 95 - protein, 902 aa, Rattus rattus [sequence omitted]

SEQ ID NO: 96 - protein, 895 aa, Papio hamadryas
MEVQLGLGRVYPRPPSKTYRGAFQNLFQSVREVIQNPGPRHPEAASAAPPGASLQQQQQQQQQETSPRQQQQQQGEDGSPQAHRRGPTGYLVLDEEQQPSQPQSAPECHPERGCVPEPGAAVAAGKGLPQQLPAPPDEDDSAAPSTLSLLGPTFPGLSSCSADLKDILSEASTMQLLQQQQQEAVSEGSSSGRAREASGAPTSSKDNYLGGTSTISDSAKELCKAVSVSMGLGVEALEHLSPGEQLRGDCMYAPVLGVPPAVRPTPCAPLAECKGSLLDDSAGKSTEDTAEYSPFKGGYTKGLEGESLGCSGSAAAGSSGTLELPSTLSLYKSGALDEAAAYQSRDYYNFPLALAGPPPPPPPPHPHARIKLENPLDYGSAWAAAAAQCRYGELASLHGAGAAGPGSGSPSAAASSSWHTLFTAEEGQLYGPCGGGGGGGGGGGGGAGEAGAVAPYGYTRPPQGLAGQEGDFTAPDVWYPGGMVSRVPYPSPTCVKSEMGPWMDSYSGPYGDMRLETARDHVLPIDYYFPPQKTCLICGDEASGCHYGALTCGSCKVFFKRAAEGKQKYLCASRNDCTIDKFRRKNCPSCRLRKCYEAGMTLGARKLKKLGNLKLQEEGEASSTTSPTEETAQKLTVSHIEGYECQPIFLNVLEAIEPGVVCAGHDNNQPDSFAALLSSLNELGERQLVHVVKWAKALPGFRNLHVDDQMAVIQYSWMGLMVFAMGWRSFTNVNSRMLYFAPDLVFNEYRMHKSRMYSQCVRMRHLSQEFGWLQITPQEFLCMKALLLFSIIPVDGLKNQKFFDELRMNYIKELDRIIACKRKNPTSCSRRFYQLTKLLDSVQPIARELHQFTFDLLIKSHMVSVDFPEMMAEIISVQVPKILSGKVKPIYFHTQ

SEQ ID NO: 97 - DNA, 2397 bp, Artificial Sequence
  ECD v.1 CAR
atgcttctcctggtgacaagccttctgctctgtgagttaccacacccagcattcctcctgattcctgaacagaagctgataagtgaggaggacttggacatccagatgacccagaccaccagcagcctgagcgccagcctgggcgatagagtgaccatcagctgcagagccagccaggacatcagcaagtacctgaactggtatcagcagaaacccgacggcaccgtgaagctgctgatctaccacaccagcagactgcacagcggcgtgcccagcagattttctggcagcggctccggcaccgactacagcctgaccatctccaacctggaacaggaagatatcgctacctacttctgtcagcaaggcaacaccctgccctacaccttcggcggaggcaccaagctggaaatcacaggcggcggaggatctggcggaggcggaagtggcggagggggatctgaagtgaaactgcaggaaagcggccctggcctggtggccccatctcagtctctgagcgtgacctgtaccgtgtccggcgtgtccctgcctgactatggcgtgtcctggatcagacagccccccagaaagggcctggaatggctgggagtgatctggggcagcgagacaacctactacaacagcgccctgaagtcccggctgaccatcatcaaggacaactccaagagccaggtgttcctgaagatgaacagcctgcagaccgacgacaccgccatctactactgcgccaagcactactactacggcggcagctacgccatggactactggggccagggcacaagcgtgaccgtgtctagcggatccgatagaagaggcggcagaatgctgaaacacaagcggcagagggacgacggggaaggcagaggcgaagtgggatctgccggcgatatgagagccgccaacctgtggcctagccccctgatgatcaagcggagcaagaagaactccctggccctgagcctgaccgccgaccagatggtgtctgccctgctggatgccgagccccccatcctgtacagcgagtacgaccccaccagacccttcagcgaggccagcatgatgggcctgctgaccaacctggccgaccgggaactggtgcacatgatcaactgggccaagcgggtgcccggcttcgtggatctgacactgcacgaccaggtgcacctgctggaatgcgcttggctggaaatcctgatgatcggcctcgtgtggcggagcatggaacaccctggcaagctgctgttcgcccccaacctgctgctggaccggaaccagggcaaatgcgtggaaggcatggtggaaatcttcgacatgctgctggccacctccagccggttccggatgatgaacctgcagggcgaagagttcgtgtgtctgaagtccatcatcctgctgaatagcggcgtgtacaccttcctgagcagcaccctgaaaagcctggaagaaaaggaccacatccaccgggtgctggacaagatcaccgacaccctgattcacctgatggccaaggccggactgaccctgcagcagcagcatcagagactggctcagctgctgctgatcctgtcccacatccggcacatgagcaacaagcggatggaacatctgtacagcatgaagtgcaagaacgtggtgcctctgttcgatctgctgctggaaatgctggacgcccacaggctgcacgccccaacatccggatccaccacgacgccagcgccgcgaccaccaacaccggcgcccaccatcgcgtcgcagcccctgtccctgcgcccagaggcgtgccggccagcggcggggggcgcagtgcacacgagggggctggacttcgcctgtgatatctacatctgggcgcccttggccgggacttgtggggtccttctcctgtcactggttatcaccctttactgcaaacggggcagaaagaaactcctgtatatattcaaacaaccatttatgagaccagtacaaactactcaagaggaagatggctgtagctgccgatttccagaagaagaagaaggaggatgtgaactgagagtgaagttcagcaggagcgcagacgcccccgcgtaccagcagggccagaaccagctctataacgagctcaatctaggacgaagagaggagtacgatgttttggacaagagacgtggccgggaccctgagatggggggaaagccgagaaggaagaaccctcaggaaggcctgtacaatgaactgcagaaagataagatggcggaggcctacagtgagattgggatgaaaggcgagcgccggaggggcaaggggcacgatggcctttaccagggtctcagtacagccaccaaggacacctacgacgcccttcacatgcaggccctgccccctcgctag

SEQ ID NO: 98 - protein, 798 aa, Artificial Sequence
  ECD v.1 CAR
MLLLVTSLLLCELPHPAFLLIPEQKLISEEDLDIQMTQTTSSLSASLGDRVTISCRASQDISKYLNWYQQKPDGTVKLLIYHTSRLHSGVPSRFSGSGSGTDYSLTISNLEQEDIATYFCQQGNTLPYTFGGGTKLEITGGGGSGGGGSGGGGSEVKLQESGPGLVAPSQSLSVTCTVSGVSLPDYGVSWIRQPPRKGLEWLGVIWGSETTYYNSALKSRLTIIKDNSKSQVFLKMNSLQTDDTAIYYCAKHYYYGGSYAMDYWGQGTSVTVSSGSDRRGGRMLKHKRQRDDGEGRGEVGSAGDMRAANLWPSPLMIKRSKKNSLALSLTADQMVSALLDAEPPILYSEYDPTRPFSEASMMGLLTNLADRELVHMINWAKRVPGFVDLTLHDQVHLLECAWLEILMIGLVWRSMEHPGKLLFAPNLLLDRNQGKCVEGMVEIFDMLLATSSRFRMMNLQGEEFVCLKSIILLNSGVYTFLSSTLKSLEEKDHIHRVLDKITDTLIHLMAKAGLTLQQQHQRLAQLLLILSHIRHMSNKRMEHLYSMKCKNVVPLFDLLLEMLDAHRLHAPTSGSTTTPAPRPPTPAPTIASQPLSLRPEACRPAAGGAVHTRGLDFACDIYIWAPLAGTCGVLLLSLVITLYCKRGRKKLLYIFKQPFMRPVQTTQEEDGCSCRFPEEEEGGCELRVKFSRSADAPAYQQGQNQLYNELNLGRREEYDVLDKRRGRDPEMGGKPRRKNPQEGLYNELQKDKMAEAYSEIGMKGERRRGKGHDGLYQGLSTATKDTYDALHMQALPPR

SEQ ID NO: 99 - DNA, 66 bp, Artificial Sequence
  CSF2RA Signal Sequence
atgcttctcctggtgacaagccttctgctctgtgagttaccacacccagcattcctcctgattcct

SEQ ID NO: 100 - protein, 22 aa, Artificial Sequence
  CSF2RA Signal Sequence
MLLLVTSLLLCELPHPAFLLIP

SEQ ID NO: 101 - DNA, 30 bp, Artificial Sequence
  cMyc tag
gaacagaagctgataagtgaggaggacttg

SEQ ID NO: 102 - protein, 10 aa, Artificial Sequence
  cMyc tag
EQKLISEEDL

SEQ ID NO: 103 - DNA, 321 bp, Artificial Sequence
  FMC63 VL
gacatccagatgacccagaccaccagcagcctgagcgccagcctgggcgatagagtgaccatcagctgcagagccagccaggacatcagcaagtacctgaactggtatcagcagaaacccgacggcaccgtgaagctgctgatctaccacaccagcagactgcacagcggcgtgcccagcagattttctggcagcggctccggcaccgactacagcctgaccatctccaacctggaacaggaagatatcgctacctacttctgtcagcaaggcaacaccctgccctacaccttcggcggaggcaccaagctggaaatcaca

SEQ ID NO: 104 - protein, 107 aa, Artificial Sequence
  FMC63 VL
DIQMTQTTSSLSASLGDRVTISCRASQDISKYLNWYQQKPDGTVKLLIYHTSRLHSGVPSRFSGSGSGTDYSLTISNLEQEDIATYFCQQGNTLPYTFGGGTKLEIT

SEQ ID NO: 105 - DNA, 44 bp, Artificial Sequence
  Linker sequence
ggcggcggaggatctggcggaggcggaagtggcggagggggatc

SEQ ID NO: 106 - protein, 15 aa, Artificial Sequence
  Linker sequence
GGGGSGGGGSGGGGS

SEQ ID NO: 107 - DNA, 360 bp, Artificial Sequence
  FMC63 VH
gaagtgaaactgcaggaaagcggccctggcctggtggccccatctcagtctctgagcgtgacctgtaccgtgtccggcgtgtccctgcctgactatggcgtgtcctggatcagacagccccccagaaagggcctggaatggctgggagtgatctggggcagcgagacaacctactacaacagcgccctgaagtcccggctgaccatcatcaaggacaactccaagagccaggtgttcctgaagatgaacagcctgcagaccgacgacaccgccatctactactgcgccaagcactactactacggcggcagctacgccatggactactggggccagggcacaagcgtgaccgtgtctagc

SEQ ID NO: 108 - protein, 120 aa, Artificial Sequence
  FMC63 VH
EVKLQESGPGLVAPSQSLSVTCTVSGVSLPDYGVSWIRQPPRKGLEWLGVIWGSETTYYNSALKSRLTIIKDNSKSQVFLKMNSLQTDDTAIYYCAKHYYYGGSYAMDYWGQGTSVTVSS

SEQ ID NO: 109 - DNA, 891 bp, Artificial Sequence
  Estrogen receptor alpha ligand binding domain
gatagaagaggcggcagaatgctgaaacacaagcggcagagggacgacggggaaggcagaggcgaagtgggatctgccggcgatatgagagccgccaacctgtggcctagccccctgatgatcaagcggagcaagaagaactccctggccctgagcctgaccgccgaccagatggtgtctgccctgctggatgccgagccccccatcctgtacagcgagtacgaccccaccagacccttcagcgaggccagcatgatgggcctgctgaccaacctggccgaccgggaactggtgcacatgatcaactgggccaagcgggtgcccggcttcgtggatctgacactgcacgaccaggtgcacctgctggaatgcgcttggctggaaatcctgatgatcggcctcgtgtggcggagcatggaacaccctggcaagctgctgttcgcccccaacctgctgctggaccggaaccagggcaaatgcgtggaaggcatggtggaaatcttcgacatgctgctggccacctccagccggttccggatgatgaacctgcagggcgaagagttcgtgtgtctgaagtccatcatcctgctgaatagcggcgtgtacaccttcctgagcagcaccctgaaaagcctggaagaaaaggaccacatccaccgggtgctggacaagatcaccgacaccctgattcacctgatggccaaggccggactgaccctgcagcagcagcatcagagactggctcagctgctgctgatcctgtcccacatccggcacatgagcaacaagcggatggaacatctgtacagcatgaagtgcaagaacgtggtgcctctgttcgatctgctgctggaaatgctggacgcccacaggctgcacgccccaacatcc

SEQ ID NO: 110 - protein, 297 aa, Artificial Sequence; identical to SEQ ID NO: 28
  Estrogen receptor alpha ligand binding domain

SEQ ID NO: 111 - DNA, 207 bp, Homo sapiens
accacgacgccagcgccgcgaccaccaacaccggcgcccaccatcgcgtcgcagcccctgtccctgcgcccagaggcgtgccggccagcggcggggggcgcagtgcacacgagggggctggacttcgcctgtgatatctacatctgggcgcccttggccgggacttgtggggtccttctcctgtcactggttatcaccctttactgc

SEQ ID NO: 112 - protein, 44 aa, Homo sapiens
TTTPAPRPPTPAPTIASQPLSLRPEACRPAAGGAVHTRGLDFAC

SEQ ID NO: 113 - DNA, 75 bp, Homo sapiens
gatatctacatctgggcgcccttggccgggacttgtggggtccttctcctgtcactggttatcaccctttactgc

SEQ ID NO: 114 - protein, 25 aa, Homo sapiens
DIYIWAPLAGTCGVLLLSLVITLYC

SEQ ID NO: 115 - DNA, 123 bp, Homo sapiens
aaacggggcagaaagaaactcctgtatatattcaaacaaccatttatgagaccagtacaaactactcaagaggaagatggctgtagctgccgatttccagaagaagaagaaggaggatgtgaa

SEQ ID NO: 116 - protein, 41 aa, Homo sapiens
KRGRKKLLYIFKQPFMRPVQTTQEEDGCSCRFPEEEEGGCE

SEQ ID NO: 117 - DNA, 339 bp, Homo sapiens
ctgagagtgaagttcagcaggagcgcagacgcccccgcgtaccagcagggccagaaccagctctataacgagctcaatctaggacgaagagaggagtacgatgttttggacaagagacgtggccgggaccctgagatggggggaaagccgagaaggaagaaccctcaggaaggcctgtacaatgaactgcagaaagataagatggcggaggcctacagtgagattgggatgaaaggcgagcgccggaggggcaaggggcacgatggcctttaccagggtctcagtacagccaccaaggacacctacgacgcccttcacatgcaggccctgccccctcgc

SEQ ID NO: 118 - protein, 113 aa, Homo sapiens; identical to SEQ ID NO: 48

SEQ ID NO: 119 - protein, 595 aa, Artificial Sequence [sequence omitted]